European Patent Application EP 4 382 606 A1, published June 12, 2024. Title: Nucleic acid construct utilizing SNARE. Applicant: 花王株式会社. The sequence listing filed with the application follows.

SEQUENCE LISTING (108 sequences)

SEQ ID NO: 1 - DNA, 663 bp, Homo sapiens
  source 1..663: mol_type = genomic DNA
atggcgattctttttgctgttgttgccagggggaccactatccttgccaaacatgcttggtgtggaggaaacttcctggaggtgacagagcagattctggctaagataccttctgaaaataacaaactaacgtactcacatggcaattatttgtttcattacatctgccaagacaggattgtatatctttgtatcactgatgatgattttgaacgttcccgagcctttaattttctgaatgagataaagaagaggttccagactacttacggttcaagagcacagacagcacttccatatgccatgaatagcgagttctcaagtgtcttagctgcacagctgaagcatcactctgagaataagggcctagacaaagtgatggagactcaagcccaagtggatgaactgaaaggaatcatggtcagaaacatagatctggtagctcagcgaggagaaagattggaattattgattgacaaaacagaaaatcttgtggattcttctgtcaccttcaaaactaccagcagaaatcttgctcgagccatgtgtatgaagaacctcaagctcactattatcatcatcatcgtatcaattgtgttcatctatatcattgtttcacctctctgtggtggatttacatggccaagctgtgtgaagaaatag

SEQ ID NO: 2 - DNA, 774 bp, Homo sapiens
  source 1..774: mol_type = genomic DNA
atggatcccctgttccagcaaacgcacaagcaggtccacgagatccagtcttgcatgggacgcctggagacggcagacaagcagtctgtgcacatagtagaaaacgaaatccaagcaagcatagaccagatattcagccgtctagaacgtctggagattttgtccagcaaggagccccctaacaaaaggcaaaatgccagacttcgggttgaccagttaaagtatgatgtccagcacctgcagactgcgctcagaaacttccagcatcggcgccatgcaagggagcagcaggagagacagcgagaagagcttctgtctcgaaccttcaccactaacgactctgacaccaccataccaatggacgaatcactgcagtttaactcctccctccagaaagttcacaacggcatggatgacctcattttagatgggcacaatattttagatggactgaggacccagagactgaccttgaaggggactcagaagaagatccttgacattgccaacatgctgggcttgtccaacacagtgatgcggctcatcgagaagcgggctttccaggacaagtactttatgatagagacaaggtctcaccatgttgcccagaatggacccgaactcctgagctcaagagatcctcctgcatcagcctcccgaagtgctgggattataggtatgagccaccaccctgacctccaaataccttttgaactcaggcttggatttgaactctggttctatcaactattagctgtgatttcagatcagtga

SEQ ID NO: 3 - DNA, 750 bp, Homo sapiens
  source 1..750: mol_type = genomic DNA
atgtctctcgaagaccccttttttgtagtccgaggcgaggtgcagaaggcggtgaacacggcccgcgggctgtaccagcgctggtgcgagctcctgcaggaaagcgcggcggtcggacgcgaggagctggactggacgaccaatgagctgcggaatggcctgcgcagcatcgagtgggacctcgaggacctggaagagaccatcggtatagtggaagccaacccaggcaagttcaagctcccagccggggacctgcaggagagaaaggtgttcgtggagcggatgcgagaggcagtccaggaaatgaaggaccatatggtcagcccaacagccgtagcatttttggagaggaataacagagagatactcgcaggcaagccagctgcccagaagtcacccagcgacctgctggatgccagcgcagtctcggccacatctcgctacatcgaggagcagcaggccacacagcagctgatcatggatgaacaggatcaacagctggagatggtgtctgggagcatccaggttctgaagcacatgtccggccgcgttggagaagagctggacgagcagggcatcatgctggatgccttcgcccaagagatggaccacacccagtcccgcatggacggggtcctcaggaagttggccaaagtatcccacatgacgagtgaccgccgacagtggtgtgccatcgccgtgctagtgggggtgcttctcctcgttctcatcttactattctctctctga

SEQ ID NO: 4 - DNA, 1008 bp, Homo sapiens
  source 1..1008: mol_type = genomic DNA
atggcggtggacatcacgctgctattccgggccagcgtcaagaccgtgaagacgcggaacaaggcgctgggagtggcggtgggcggcggggtcgatggcagccgggacgagctgttccgccggagcccccggcccaagggcgacttctccagccgggcccgcgaagtgatttctcacattggcaaactgagagattttcttctggaacacaggaaagattatattaatgcttatagccataccatgtctgaatatgggaggatgacagacacagaacgagaccagatagaccaggatgcccagatattcatgaggacctgttcagaagcaattcagcaactacgaacagaagctcacaaggagatacattcccagcaagtgaaggagcacaggaccgctgttttggatttcattgaagattacttgaaaagagtatgtaaactttactcagaacagagagccatccgagttaaaagagtggtggataagaaaagattatctaagctggaaccagaaccaaatacaaagacaagagaatccacatcttctgagaaagtttcacagagtccttcaaaagactctgaagaaaaccctgccactgaagaacgtccagaaaaaattttggctgaaacacaacctgaattgggaacgtggggagatggcaaaggcgaagatgagttatccccagaagaaatacaaatgtttgaacaggaaaatcagcgactaattggtgaaatgaacagcttgtttgatgaagtgaggcaaatcgaagggagagtggttgagatttccagactccaagagatattcacggaaaaggttttgcaacaggaagctgagattgacagcattcaccagttagttgtgggggcaactgaaaatatcaaggaaggcaacgaagacataagagaggccattaaaaacaacgctggcttccgcgtgtggatcctcttcttcctcgtgatgtgctccttctccttgctcttcctcgactggtacgacagctag

SEQ ID NO: 5 - DNA, 816 bp, Homo sapiens
  source 1..816: mol_type = genomic DNA
atggcggctccccaagacgtccacgtccggatctgtaaccaagagattgtcaaatttgacctggaggtgaaggcgcttattcaggatatccgtgattgttcaggacccttaagtgctcttactgaactgaatactaaagtaaaagagaaatttcaacagttgcgtcacagaatacagccagttctctatcaaagggcatttatttggactgcttccacatttttttttaagctaacttattccctgacagacttttcttcaactcagcatgacttcaactctccaactacacctgttaccttcagtgacctggagcagttggctaaagagcaagacaaagaatcagagaaacaacttctactccaggaagtggagaatcacaaaaagcagatgctcagcaatcaggcctcatggaggaaagctaatctcacctgcaaaattgcaatcgacaatctagagaaagcagaacttcttcagggaggagatctcttaaggcaaaggaaaaccaccaaagagagcctggcccagacatccagtaccatcactgagagcctcatggggatcagcaggatgatggcccagcaggtccagcagagcgaggaggccatgcagtctctagtcacttcttcacgaacgatcctggatgcaaatgaagaatttaagtccatgtcgggcaccatccagctgggccggaagcttatcacaaaatacaatcgccgggagctgacggacaagcttctcatcttccttgcgctagccctgtttcttgctacggtcctctatattgtgaaaaagcggctctttccatttttgtga

SEQ ID NO: 6 - DNA, 786 bp, Homo sapiens
  source 1..786: mol_type = genomic DNA
atgtcttacactccaggagttggtggtgaccccgcccagttggcccagaggatctcttctaacatccagaagatcacacagtgttctgtggaaatacaaagaactctgaatcaacttggaacacctcaagattcacctgaattgaggcaacagttgcaacagaagcagcagtatactaaccagcttgccaaagaaacagataagtacattaaagagtttggatctctgcccaccacccccagtgaacagcgtcaaaggaaaatacagaaggatcgcttagtggcagagttcacaacatcactgacaaacttccagaaggtccagaggcaggctgctgagcgagagaaagagtttgttgctcgagtaagagccagttccagagtgtctggcagttttcctgaggacagctcaaaagaaaggaatcttgtatcctgggaaagccaaactcaacctcaagtgcaggtgcaggatgaagaaattacagaggatgacctccgtcttattcatgagagagaatcttctatcaggcaacttgaagctgatattatggatattaatgaaatatttaaagatttgggaatgatgattcatgaacaaggagatgtaatagatagcatagaagccaatgtggaaaatgcagaggtgcacgttcagcaagcaaatcagcagctgtcaagggcagcagattatcagcgcaaatccagaaaaaccctgtgcatcatcattcttatccttgtcattggagttgcgattatcagtctcatcatatggggattgaaccactga

SEQ ID NO: 7 - DNA, 675 bp, Homo sapiens
  source 1..675: mol_type = genomic DNA
atgtcgtccgacttcgaaggttacgagcaggacttcgcggtgctcactgcagagatcaccagcaagattgcgagggtcccacgactcccgcctgatgaaaagaaacagatggttgcaaatgtggagaaacagcttgaagaagcgaaagaactgcttgaacagatggatttggaagtccgagagataccaccccaaagtcgagggatgtacagcaacagaatgagaagctacaaacaagaaatgggaaaactcgaaacagattttaaaaggtcacggatcgcctacagtgacgaagtacggaatgagctcctgggggatgatgggaattcctcagagaaccagttgataaaattacgtgaagagagggcacatctgctcgataacacagagaggctggaaaggtcatctcggagactagaggctggataccaaatagcagtggaaaccgagcaaattggtcaggagatgttggaaaaccttagtcatgacagagaaaagatacagcgagcacgtgaaagacttcgggaaacagatgctaatttgggaaaaagctccaggattctgacagggatgttgcgaagaatcatccagaaccgcatcctgctcgtcatcctagggatcatcgtggtcatcaccatcctgatggcgatcactttttctgtcagaagacactga

SEQ ID NO: 8 - DNA, 978 bp, Homo sapiens
  source 1..978: mol_type = genomic DNA
atggccaccaggcgtttaaccgacgctttcttgttgttgcggaataattccatccaaaaccggcagctgttagccgagcaagtgagtagtcacatcacctccagccctctgcattcacgtagcattgctgcggagctggacgagcttgctgatgaccgtatggcactggtgtcaggcatcagcttagatccagaagcagcgattggtgtgacaaaacggccacctcctaagtgggtggatggagtggatgaaattcagtatgatgttggccggattaagcagaagatgaaagaattggccagccttcatgacaagcatttaaacagacccaccctggatgacagcagcgaagaggaacatgccattgagataactacccaagagatcactcagctcttccacaggtgccagcgtgccgtgcaggccctgccgagccgggcccgggcctgctccgagcaggaggggcggctgcttgggaacgtggtggcctcgctggcgcaggccctgcaggaactctccaccagcttccggcacgcacagtcaggctacctcaaacgcatgaagaatcgagaggaaagatcccagcattttttcgacacatcagtaccactaatggatgatggagacgataacactctttaccatcggggttttacagaggaccagttagttctggtggagcagaacacactgatggtggaagagcgggaacgagagattcgccagattgtacagtccatttctgacctgaatgaaatattcagggacttaggggcgatgattgtagaacagggtacagtccttgacagaattgactataacgttgaacagtcctgtatcaaaactgaagatggtttgaaacagcttcacaaggcagaacagtatcaaaagaagaatcggaagatgcttgtgattttaatattatttgtcatcatcattgtgctcattgttgtcctcgttggcgtgaagtctcgataa

SEQ ID NO: 9 - DNA, 1068 bp, Homo sapiens
  source 1..1068: mol_type = genomic DNA
atgatcccgcggaaacgctacgggtctaagaacacggatcagggtgtctacctgggtctctcaaagacacaggtcctgtcccctgcaactgctggcagtagcagcagcgacatcgcccctctgccccccccagtgaccctcgtccctccccctcccgacaccatgtcctgccgggatcggacccaggagtttctgtctgcctgcaagtcgctgcagacccgtcagaatggaatccagacaaataagccagctttgcgtgctgtccgacaacgcagtgaattcaccctcatggccaagcgcattgggaaagaccttagcaacacatttgccaagctggagaagctgacaatcttggcaaagcgcaagtccctctttgatgataaagcagtggaaattgaagagctaacatatatcatcaaacaggacatcaatagcctcaacaaacaaattgctcagctccaggatttcgtgagagccaagggcagccagagtggccggcacctgcagacccactccaacaccattgtggtctccttgcagtcgaaactggcttctatgtccaatgacttcaaatcggttttagaagtgaggacagagaacctgaagcagcagaggagccggagagagcagttctcccgggcacctgtgtcagccctgccccttgcccctaaccacctgggcggtggtgctgtggttctgggggcagagtcccatgcctccaaggatgtcgccatcgacatgatggactctcggaccagccagcagctgcagctcattgacgagcaggattcctacatccagagtcgggcagacaccatgcagaacattgagtcgacaattgttgagttgggctccatctttcagcagttggcacacatggttaaggaacaggaggaaaccattcagaggatcgacgagaacgtgctaggagcccagctggacgttgaggccgcccattcagagatcctcaagtacttccagtctgtcacctccaaccggtggctcatggtcaaaatcttcctcatcctcattgtcttcttcatcatctttgtggtcttccttgcttga

SEQ ID NO: 10 - protein, 220 aa, Homo sapiens
MAILFAVVARGTTILAKHAWCGGNFLEVTEQILAKIPSENNKLTYSHGNYLFHYICQDRIVYLCITDDDFERSRAFNFLNEIKKRFQTTYGSRAQTALPYAMNSEFSSVLAAQLKHHSENKGLDKVMETQAQVDELKGIMVRNIDLVAQRGERLELLIDKTENLVDSSVTFKTTSRNLARAMCMKNLKLTIIIIIVSIVFIYIIVSPLCGGFTWPSCVKK

SEQ ID NO: 11 - protein, 257 aa, Homo sapiens
MDPLFQQTHKQVHEIQSCMGRLETADKQSVHIVENEIQASIDQIFSRLERLEILSSKEPPNKRQNARLRVDQLKYDVQHLQTALRNFQHRRHAREQQERQREELLSRTFTTNDSDTTIPMDESLQFNSSLQKVHNGMDDLILDGHNILDGLRTQRLTLKGTQKKILDIANMLGLSNTVMRLIEKRAFQDKYFMIETRSHHVAQNGPELLSSRDPPASASRSAGIIGMSHHPDLQIPFELRLGFELWFYQLLAVISDQ

SEQ ID NO: 12 - protein, 249 aa, Homo sapiens
MSLEDPFFVVRGEVQKAVNTARGLYQRWCELLQESAAVGREELDWTTNELRNGLRSIEWDLEDLEETIGIVEANPGKFKLPAGDLQERKVFVERMREAVQEMKDHMVSPTAVAFLERNNREILAGKPAAQKSPSDLLDASAVSATSRYIEEQQATQQLIMDEQDQQLEMVSGSIQVLKHMSGRVGEELDEQGIMLDAFAQEMDHTQSRMDGVLRKLAKVSHMTSDRRQWCAIAVLVGVLLLVLILLFSL

SEQ ID NO: 13 - protein, 335 aa, Homo sapiens
MAVDITLLFRASVKTVKTRNKALGVAVGGGVDGSRDELFRRSPRPKGDFSSRAREVISHIGKLRDFLLEHRKDYINAYSHTMSEYGRMTDTERDQIDQDAQIFMRTCSEAIQQLRTEAHKEIHSQQVKEHRTAVLDFIEDYLKRVCKLYSEQRAIRVKRVVDKKRLSKLEPEPNTKTRESTSSEKVSQSPSKDSEENPATEERPEKILAETQPELGTWGDGKGEDELSPEEIQMFEQENQRLIGEMNSLFDEVRQIEGRVVEISRLQEIFTEKVLQQEAEIDSIHQLVVGATENIKEGNEDIREAIKNNAGFRVWILFFLVMCSFSLLFLDWYDS

SEQ ID NO: 14 - protein, 271 aa, Homo sapiens
MAAPQDVHVRICNQEIVKFDLEVKALIQDIRDCSGPLSALTELNTKVKEKFQQLRHRIQPVLYQRAFIWTASTFFFKLTYSLTDFSSTQHDFNSPTTPVTFSDLEQLAKEQDKESEKQLLLQEVENHKKQMLSNQASWRKANLTCKIAIDNLEKAELLQGGDLLRQRKTTKESLAQTSSTITESLMGISRMMAQQVQQSEEAMQSLVTSSRTILDANEEFKSMSGTIQLGRKLITKYNRRELTDKLLIFLALALFLATVLYIVKKRLFPFL

SEQ ID NO: 15 - protein, 261 aa, Homo sapiens
MSYTPGVGGDPAQLAQRISSNIQKITQCSVEIQRTLNQLGTPQDSPELRQQLQQKQQYTNQLAKETDKYIKEFGSLPTTPSEQRQRKIQKDRLVAEFTTSLTNFQKVQRQAAEREKEFVARVRASSRVSGSFPEDSSKERNLVSWESQTQPQVQVQDEEITEDDLRLIHERESSIRQLEADIMDINEIFKDLGMMIHEQGDVIDSIEANVENAEVHVQQANQQLSRAADYQRKSRKTLCIIILILVIGVAIISLIIWGLNH

SEQ ID NO: 16 - protein, 224 aa, Homo sapiens
MSSDFEGYEQDFAVLTAEITSKIARVPRLPPDEKKQMVANVEKQLEEAKELLEQMDLEVREIPPQSRGMYSNRMRSYKQEMGKLETDFKRSRIAYSDEVRNELLGDDGNSSENQLIKLREERAHLLDNTERLERSSRRLEAGYQIAVETEQIGQEMLENLSHDREKIQRARERLRETDANLGKSSRILTGMLRRIIQNRILLVILGIIVVITILMAITFSVRRH

SEQ ID NO: 17 - protein, 325 aa, Homo sapiens
MATRRLTDAFLLLRNNSIQNRQLLAEQVSSHITSSPLHSRSIAAELDELADDRMALVSGISLDPEAAIGVTKRPPPKWVDGVDEIQYDVGRIKQKMKELASLHDKHLNRPTLDDSSEEEHAIEITTQEITQLFHRCQRAVQALPSRARACSEQEGRLLGNVVASLAQALQELSTSFRHAQSGYLKRMKNREERSQHFFDTSVPLMDDGDDNTLYHRGFTEDQLVLVEQNTLMVEEREREIRQIVQSISDLNEIFRDLGAMIVEQGTVLDRIDYNVEQSCIKTEDGLKQLHKAEQYQKKNRKMLVILILFVIIIVLIVVLVGVKSR

SEQ ID NO: 18 - protein, 355 aa, Homo sapiens
MIPRKRYGSKNTDQGVYLGLSKTQVLSPATAGSSSSDIAPLPPPVTLVPPPPDTMSCRDRTQEFLSACKSLQTRQNGIQTNKPALRAVRQRSEFTLMAKRIGKDLSNTFAKLEKLTILAKRKSLFDDKAVEIEELTYIIKQDINSLNKQIAQLQDFVRAKGSQSGRHLQTHSNTIVVSLQSKLASMSNDFKSVLEVRTENLKQQRSRREQFSRAPVSALPLAPNHLGGGAVVLGAESHASKDVAIDMMDSRTSQQLQLIDEQDSYIQSRADTMQNIESTIVELGSIFQQLAHMVKEQEETIQRIDENVLGAQLDVEAAHSEILKYFQSVTSNRWLMVKIFLILIVFFIIFVVFLA

SEQ ID NO: 19 - DNA, 45 bp, synthetic construct
  source 1..45: mol_type = other DNA; note = linker
ggcggcggaggatctggcggaggtggaagcggaggcggaggaagt

SEQ ID NO: 20 - protein, 15 aa, synthetic construct
  source 1..15: note = linker
GGGGSGGGGSGGGGS

SEQ ID NO: 21 - DNA, 15 bp, synthetic construct
  source 1..15: mol_type = other DNA; note = proprotein convertase (e.g., furin) recognition sequence
agaagggccagaaga

SEQ ID NO: 22 - protein, 5 aa, synthetic construct
  source 1..5: note = proprotein convertase (e.g., furin) recognition sequence
RRARR

SEQ ID NO: 23 - DNA, 1161 bp, Gallus gallus
  source 1..1161: mol_type = genomic DNA
atgggctccatcggcgcagcaagcatggaattttgttttgatgtattcaaggagctcaaagtccaccatgccaatgagaacatcttctactgccccattgccatcatgtcagctctagccatggtatacctgggtgcaaaagacagcaccaggacacagataaataaggttgttcgctttgataaacttccaggattcggagacagtattgaagctcagtgtggcacatctgtaaacgttcactcttcacttagagacatcctcaaccaaatcaccaaaccaaatgatgtttattcgttcagccttgccagtagactttatgctgaagagagatacccaatcctgccagaatacttgcagtgtgtgaaggaactgtatagaggaggcttggaacctatcaactttcaaacagctgcagatcaagccagagagctcatcaattcctgggtagaaagtcagacaaatggaattatcagaaatgtccttcagccaagctccgtggattctcaaactgcaatggttctggttaatgccattgtcttcaaaggactgtgggagaaaacatttaaggatgaagacacacaagcaatgcctttcagagtgactgagcaagaaagcaaacctgtgcagatgatgtaccagattggtttatttagagtggcatcaatggcttctgagaaaatgaagatcctggagcttccatttgccagtgggacaatgagcatgttggtgctgttgcctgatgaagtctcaggccttgagcagcttgagagtataatcaactttgaaaaactgactgaatggaccagttctaatgttatggaagagaggaagatcaaagtgtacttacctcgcatgaagatggaggaaaaatacaacctcacatctgtcttaatggctatgggcattactgacgtgtttagctcttcagccaatctgtctggcatctcctcagcagagagcctgaagatatctcaagctgtccatgcagcacatgcagaaatcaatgaagcaggcagagaggtggtagggtcagcagaggctggagtggatgctgcaagcgtctctgaagaatttagggctgaccatccattcctcttctgtatcaagcacatcgcaaccaacgccgttctcttctttggcagatgtgtttccccttaa

SEQ ID NO: 24 - protein, 386 aa, Gallus gallus
MGSIGAASMEFCFDVFKELKVHHANENIFYCPIAIMSALAMVYLGAKDSTRTQINKVVRFDKLPGFGDSIEAQCGTSVNVHSSLRDILNQITKPNDVYSFSLASRLYAEERYPILPEYLQCVKELYRGGLEPINFQTAADQARELINSWVESQTNGIIRNVLQPSSVDSQTAMVLVNAIVFKGLWEKTFKDEDTQAMPFRVTEQESKPVQMMYQIGLFRVASMASEKMKILELPFASGTMSMLVLLPDEVSGLEQLESIINFEKLTEWTSSNVMEERKIKVYLPRMKMEEKYNLTSVLMAMGITDVFSSSANLSGISSAESLKISQAVHAAHAEINEAGREVVGSAEAGVDAASVSEEFRADHPFLFCIKHIATNAVLFFGRCVSP

SEQ ID NO: 25 - protein, 621 aa, synthetic construct
  source 1..621: note = VAMP7-OVA
MAILFAVVARGTTILAKHAWCGGNFLEVTEQILAKIPSENNKLTYSHGNYLFHYICQDRIVYLCITDDDFERSRAFNFLNEIKKRFQTTYGSRAQTALPYAMNSEFSSVLAAQLKHHSENKGLDKVMETQAQVDELKGIMVRNIDLVAQRGERLELLIDKTENLVDSSVTFKTTSRNLARAMCMKNLKLTIIIIIVSIVFIYIIVSPLCGGFTWPSCVKKSGGGGSGGGGSGGGGSGSIGAASMEFCFDVFKELKVHHANENIFYCPIAIMSALAMVYLGAKDSTRTQINKVVRFDKLPGFGDSIEAQCGTSVNVHSSLRDILNQITKPNDVYSFSLASRLYAEERYPILPEYLQCVKELYRGGLEPINFQTAADQARELINSWVESQTNGIIRNVLQPSSVDSQTAMVLVNAIVFKGLWEKTFKDEDTQAMPFRVTEQESKPVQMMYQIGLFRVASMASEKMKILELPFASGTMSMLVLLPDEVSGLEQLESIINFEKLTEWTSSNVMEERKIKVYLPRMKMEEKYNLTSVLMAMGITDVFSSSANLSGISSAESLKISQAVHAAHAEINEAGREVVGSAEAGVDAASVSEEFRADHPFLFCIKHIATNAVLFFGRCVSP

SEQ ID NO: 26 - protein, 657 aa, synthetic construct
  source 1..657: note = GOSR2-OVA
MDPLFQQTHKQVHEIQSCMGRLETADKQSVHIVENEIQASIDQIFSRLERLEILSSKEPPNKRQNARLRVDQLKYDVQHLQTALRNFQHRRHAREQQERQREELLSRTFTTNDSDTTIPMDESLQFNSSLQKVHNGMDDLILDGHNILDGLRTQRLTLKGTQKKILDIANMLGLSNTVMRLIEKRAFQDKYFMIETRSHHVAQNGPELLSSRDPPASASRSAGIIGMSHHPDLQIPFELRLGFELWFYQLLAVISDQGGGGSGGGGSGGGGSGSIGAASMEFCFDVFKELKVHHANENIFYCPIAIMSALAMVYLGAKDSTRTQINKVVRFDKLPGFGDSIEAQCGTSVNVHSSLRDILNQITKPNDVYSFSLASRLYAEERYPILPEYLQCVKELYRGGLEPINFQTAADQARELINSWVESQTNGIIRNVLQPSSVDSQTAMVLVNAIVFKGLWEKTFKDEDTQAMPFRVTEQESKPVQMMYQIGLFRVASMASEKMKILELPFASGTMSMLVLLPDEVSGLEQLESIINFEKLTEWTSSNVMEERKIKVYLPRMKMEEKYNLTSVLMAMGITDVFSSSANLSGISSAESLKISQAVHAAHAEINEAGREVVGSAEAGVDAASVSEEFRADHPFLFCIKHIATNAVLFFGRCVSP

SEQ ID NO: 27 - protein, 649 aa, synthetic construct
  source 1..649: note = STX10-OVA
MSLEDPFFVVRGEVQKAVNTARGLYQRWCELLQESAAVGREELDWTTNELRNGLRSIEWDLEDLEETIGIVEANPGKFKLPAGDLQERKVFVERMREAVQEMKDHMVSPTAVAFLERNNREILAGKPAAQKSPSDLLDASAVSATSRYIEEQQATQQLIMDEQDQQLEMVSGSIQVLKHMSGRVGEELDEQGIMLDAFAQEMDHTQSRMDGVLRKLAKVSHMTSDRRQWCAIAVLVGVLLLVLILLFSLGGGGSGGGGSGGGGSGSIGAASMEFCFDVFKELKVHHANENIFYCPIAIMSALAMVYLGAKDSTRTQINKVVRFDKLPGFGDSIEAQCGTSVNVHSSLRDILNQITKPNDVYSFSLASRLYAEERYPILPEYLQCVKELYRGGLEPINFQTAADQARELINSWVESQTNGIIRNVLQPSSVDSQTAMVLVNAIVFKGLWEKTFKDEDTQAMPFRVTEQESKPVQMMYQIGLFRVASMASEKMKILELPFASGTMSMLVLLPDEVSGLEQLESIINFEKLTEWTSSNVMEERKIKVYLPRMKMEEKYNLTSVLMAMGITDVFSSSANLSGISSAESLKISQAVHAAHAEINEAGREVVGSAEAGVDAASVSEEFRADHPFLFCIKHIATNAVLFFGRCVSP

SEQ ID NO: 28 - protein, 735 aa, synthetic construct
  source 1..735: note = STX18-OVA
MAVDITLLFRASVKTVKTRNKALGVAVGGGVDGSRDELFRRSPRPKGDFSSRAREVISHIGKLRDFLLEHRKDYINAYSHTMSEYGRMTDTERDQIDQDAQIFMRTCSEAIQQLRTEAHKEIHSQQVKEHRTAVLDFIEDYLKRVCKLYSEQRAIRVKRVVDKKRLSKLEPEPNTKTRESTSSEKVSQSPSKDSEENPATEERPEKILAETQPELGTWGDGKGEDELSPEEIQMFEQENQRLIGEMNSLFDEVRQIEGRVVEISRLQEIFTEKVLQQEAEIDSIHQLVVGATENIKEGNEDIREAIKNNAGFRVWILFFLVMCSFSLLFLDWYDSGGGGSGGGGSGGGGSGSIGAASMEFCFDVFKELKVHHANENIFYCPIAIMSALAMVYLGAKDSTRTQINKVVRFDKLPGFGDSIEAQCGTSVNVHSSLRDILNQITKPNDVYSFSLASRLYAEERYPILPEYLQCVKELYRGGLEPINFQTAADQARELINSWVESQTNGIIRNVLQPSSVDSQTAMVLVNAIVFKGLWEKTFKDEDTQAMPFRVTEQESKPVQMMYQIGLFRVASMASEKMKILELPFASGTMSMLVLLPDEVSGLEQLESIINFEKLTEWTSSNVMEERKIKVYLPRMKMEEKYNLTSVLMAMGITDVFSSSANLSGISSAESLKISQAVHAAHAEINEAGREVVGSAEAGVDAASVSEEFRADHPFLFCIKHIATNAVLFFGRCVSP

SEQ ID NO: 29 - protein, 671 aa, synthetic construct
  source 1..671: note = BNIP1-OVA
MAAPQDVHVRICNQEIVKFDLEVKALIQDIRDCSGPLSALTELNTKVKEKFQQLRHRIQPVLYQRAFIWTASTFFFKLTYSLTDFSSTQHDFNSPTTPVTFSDLEQLAKEQDKESEKQLLLQEVENHKKQMLSNQASWRKANLTCKIAIDNLEKAELLQGGDLLRQRKTTKESLAQTSSTITESLMGISRMMAQQVQQSEEAMQSLVTSSRTILDANEEFKSMSGTIQLGRKLITKYNRRELTDKLLIFLALALFLATVLYIVKKRLFPFLGGGGSGGGGSGGGGSGSIGAASMEFCFDVFKELKVHHANENIFYCPIAIMSALAMVYLGAKDSTRTQINKVVRFDKLPGFGDSIEAQCGTSVNVHSSLRDILNQITKPNDVYSFSLASRLYAEERYPILPEYLQCVKELYRGGLEPINFQTAADQARELINSWVESQTNGIIRNVLQPSSVDSQTAMVLVNAIVFKGLWEKTFKDEDTQAMPFRVTEQESKPVQMMYQIGLFRVASMASEKMKILELPFASGTMSMLVLLPDEVSGLEQLESIINFEKLTEWTSSNVMEERKIKVYLPRMKMEEKYNLTSVLMAMGITDVFSSSANLSGISSAESLKISQAVHAAHAEINEAGREVVGSAEAGVDAASVSEEFRADHPFLFCIKHIATNAVLFFGRCVSP

SEQ ID NO: 30 - protein, 661 aa, synthetic construct
  source 1..661: note = STX7-OVA
MSYTPGVGGDPAQLAQRISSNIQKITQCSVEIQRTLNQLGTPQDSPELRQQLQQKQQYTNQLAKETDKYIKEFGSLPTTPSEQRQRKIQKDRLVAEFTTSLTNFQKVQRQAAEREKEFVARVRASSRVSGSFPEDSSKERNLVSWESQTQPQVQVQDEEITEDDLRLIHERESSIRQLEADIMDINEIFKDLGMMIHEQGDVIDSIEANVENAEVHVQQANQQLSRAADYQRKSRKTLCIIILILVIGVAIISLIIWGLNHGGGGSGGGGSGGGGSGSIGAASMEFCFDVFKELKVHHANENIFYCPIAIMSALAMVYLGAKDSTRTQINKVVRFDKLPGFGDSIEAQCGTSVNVHSSLRDILNQITKPNDVYSFSLASRLYAEERYPILPEYLQCVKELYRGGLEPINFQTAADQARELINSWVESQTNGIIRNVLQPSSVDSQTAMVLVNAIVFKGLWEKTFKDEDTQAMPFRVTEQESKPVQMMYQIGLFRVASMASEKMKILELPFASGTMSMLVLLPDEVSGLEQLESIINFEKLTEWTSSNVMEERKIKVYLPRMKMEEKYNLTSVLMAMGITDVFSSSANLSGISSAESLKISQAVHAAHAEINEAGREVVGSAEAGVDAASVSEEFRADHPFLFCIKHIATNAVLFFGRCVSP

SEQ ID NO: 31 - protein, 624 aa, synthetic construct
  source 1..624: note = VTI1A-OVA
MSSDFEGYEQDFAVLTAEITSKIARVPRLPPDEKKQMVANVEKQLEEAKELLEQMDLEVREIPPQSRGMYSNRMRSYKQEMGKLETDFKRSRIAYSDEVRNELLGDDGNSSENQLIKLREERAHLLDNTERLERSSRRLEAGYQIAVETEQIGQEMLENLSHDREKIQRARERLRETDANLGKSSRILTGMLRRIIQNRILLVILGIIVVITILMAITFSVRRHGGGGSGGGGSGGGGSGSIGAASMEFCFDVFKELKVHHANENIFYCPIAIMSALAMVYLGAKDSTRTQINKVVRFDKLPGFGDSIEAQCGTSVNVHSSLRDILNQITKPNDVYSFSLASRLYAEERYPILPEYLQCVKELYRGGLEPINFQTAADQARELINSWVESQTNGIIRNVLQPSSVDSQTAMVLVNAIVFKGLWEKTFKDEDTQAMPFRVTEQESKPVQMMYQIGLFRVASMASEKMKILELPFASGTMSMLVLLPDEVSGLEQLESIINFEKLTEWTSSNVMEERKIKVYLPRMKMEEKYNLTSVLMAMGITDVFSSSANLSGISSAESLKISQAVHAAHAEINEAGREVVGSAEAGVDAASVSEEFRADHPFLFCIKHIATNAVLFFGRCVSP

SEQ ID NO: 32 - protein, 725 aa, synthetic construct
  source 1..725: note = STX16-OVA
MATRRLTDAFLLLRNNSIQNRQLLAEQVSSHITSSPLHSRSIAAELDELADDRMALVSGISLDPEAAIGVTKRPPPKWVDGVDEIQYDVGRIKQKMKELASLHDKHLNRPTLDDSSEEEHAIEITTQEITQLFHRCQRAVQALPSRARACSEQEGRLLGNVVASLAQALQELSTSFRHAQSGYLKRMKNREERSQHFFDTSVPLMDDGDDNTLYHRGFTEDQLVLVEQNTLMVEEREREIRQIVQSISDLNEIFRDLGAMIVEQGTVLDRIDYNVEQSCIKTEDGLKQLHKAEQYQKKNRKMLVILILFVIIIVLIVVLVGVKSRGGGGSGGGGSGGGGSGSIGAASMEFCFDVFKELKVHHANENIFYCPIAIMSALAMVYLGAKDSTRTQINKVVRFDKLPGFGDSIEAQCGTSVNVHSSLRDILNQITKPNDVYSFSLASRLYAEERYPILPEYLQCVKELYRGGLEPINFQTAADQARELINSWVESQTNGIIRNVLQPSSVDSQTAMVLVNAIVFKGLWEKTFKDEDTQAMPFRVTEQESKPVQMMYQIGLFRVASMASEKMKILELPFASGTMSMLVLLPDEVSGLEQLESIINFEKLTEWTSSNVMEERKIKVYLPRMKMEEKYNLTSVLMAMGITDVFSSSANLSGISSAESLKISQAVHAAHAEINEAGREVVGSAEAGVDAASVSEEFRADHPFLFCIKHIATNAVLFFGRCVSP

SEQ ID NO: 33 - protein, 755 aa, synthetic construct
  source 1..755: note = STX5-OVA
MIPRKRYGSKNTDQGVYLGLSKTQVLSPATAGSSSSDIAPLPPPVTLVPPPPDTMSCRDRTQEFLSACKSLQTRQNGIQTNKPALRAVRQRSEFTLMAKRIGKDLSNTFAKLEKLTILAKRKSLFDDKAVEIEELTYIIKQDINSLNKQIAQLQDFVRAKGSQSGRHLQTHSNTIVVSLQSKLASMSNDFKSVLEVRTENLKQQRSRREQFSRAPVSALPLAPNHLGGGAVVLGAESHASKDVAIDMMDSRTSQQLQLIDEQDSYIQSRADTMQNIESTIVELGSIFQQLAHMVKEQEETIQRIDENVLGAQLDVEAAHSEILKYFQSVTSNRWLMVKIFLILIVFFIIFVVFLAGGGGSGGGGSGGGGSGSIGAASMEFCFDVFKELKVHHANENIFYCPIAIMSALAMVYLGAKDSTRTQINKVVRFDKLPGFGDSIEAQCGTSVNVHSSLRDILNQITKPNDVYSFSLASRLYAEERYPILPEYLQCVKELYRGGLEPINFQTAADQARELINSWVESQTNGIIRNVLQPSSVDSQTAMVLVNAIVFKGLWEKTFKDEDTQAMPFRVTEQESKPVQMMYQIGLFRVASMASEKMKILELPFASGTMSMLVLLPDEVSGLEQLESIINFEKLTEWTSSNVMEERKIKVYLPRMKMEEKYNLTSVLMAMGITDVFSSSANLSGISSAESLKISQAVHAAHAEINEAGREVVGSAEAGVDAASVSEEFRADHPFLFCIKHIATNAVLFFGRCVSP

SEQ ID NO: 34 - protein, 655 aa, synthetic construct
  source 1..655: note = STX6-OVA
MSMEDPFFVVKGEVQKAVNTAQGLFQRWTELLQDPSTATREEIDWTTNELRNNLRSIEWDLEDLDETISIVEANPRKFNLDATELSIRKAFITSTRQVVRDMKDQMSTSSVQALAERKNRQALLGDSGSQNWSTGTTDKYGRLDRELQRANSHFIEEQQAQQQLIVEQQDEQLELVSGSIGVLKNMSQRIGGELEEQAVMLEDFSHELESTQSRLDNVMKKLAKVSHMTSDRRQWCAIAILFAVLLVVLILFLVLGGGGSGGGGSGGGGSGSIGAASMEFCFDVFKELKVHHANENIFYCPIAIMSALAMVYLGAKDSTRTQINKVVRFDKLPGFGDSIEAQCGTSVNVHSSLRDILNQITKPNDVYSFSLASRLYAEERYPILPEYLQCVKELYRGGLEPINFQTAADQARELINSWVESQTNGIIRNVLQPSSVDSQTAMVLVNAIVFKGLWEKTFKDEDTQAMPFRVTEQESKPVQMMYQIGLFRVASMASEKMKILELPFASGTMSMLVLLPDEVSGLEQLESIINFEKLTEWTSSNVMEERKIKVYLPRMKMEEKYNLTSVLMAMGITDVFSSSANLSGISSAESLKISQAVHAAHAEINEAGREVVGSAEAGVDAASVSEEFRADHPFLFCIKHIATNAVLFFGRCVSP

SEQ ID NO: 35 - protein, 636 aa, synthetic construct
  source 1..636: note = STX8-OVA
MAPDPWFSTYDSTCQIAQEIAEKIQQRNQYERKGEKAPKLTVTIRALLQNLKEKIALLKDLLLRAVSTHQITQLEGDRRQNLLDDLVTRERLLLASFKNEGAEPDLIRSSLMSEEAKRGAPNPWLFEEPEETRGLGFDEIRQQQQKIIQEQDAGLDALSSIISRQKQMGQEIGNELDEQNEIIDDLANLVENTDEKLRNETRRVNMVDRKSASCGMIMVILLLLVAIVVVAVWPTNGGGGSGGGGSGGGGSGSIGAASMEFCFDVFKELKVHHANENIFYCPIAIMSALAMVYLGAKDSTRTQINKVVRFDKLPGFGDSIEAQCGTSVNVHSSLRDILNQITKPNDVYSFSLASRLYAEERYPILPEYLQCVKELYRGGLEPINFQTAADQARELINSWVESQTNGIIRNVLQPSSVDSQTAMVLVNAIVFKGLWEKTFKDEDTQAMPFRVTEQESKPVQMMYQIGLFRVASMASEKMKILELPFASGTMSMLVLLPDEVSGLEQLESIINFEKLTEWTSSNVMEERKIKVYLPRMKMEEKYNLTSVLMAMGITDVFSSSANLSGISSAESLKISQAVHAAHAEINEAGREVVGSAEAGVDAASVSEEFRADHPFLFCIKHIATNAVLFFGRCVSP

SEQ ID NO: 36 - protein, 676 aa, synthetic construct
  source 1..676: note = STX12-OVA
MSYGPLDMYRNPGPSGPQLRDFSSIIQTCSGNIQRISQATAQIKNLMSQLGTKQDSSKLQENLQQLQHSTNQLAKETNELLKELGSLPLPLSTSEQRQQRLQKERLMNDFSAALNNFQAVQRRVSEKEKESIARARAGSRLSAEERQREEQLVSFDSHEEWNQMQSQEDEVAITEQDLELIKERETAIRQLEADILDVNQIFKDLAMMIHDQGDLIDSIEANVESSEVHVERATEQLQRAAYYQKKSRKKMCILVLVLSVIILILGLIIWLVYKTKGGGGSGGGGSGGGGSGSIGAASMEFCFDVFKELKVHHANENIFYCPIAIMSALAMVYLGAKDSTRTQINKVVRFDKLPGFGDSIEAQCGTSVNVHSSLRDILNQITKPNDVYSFSLASRLYAEERYPILPEYLQCVKELYRGGLEPINFQTAADQARELINSWVESQTNGIIRNVLQPSSVDSQTAMVLVNAIVFKGLWEKTFKDEDTQAMPFRVTEQESKPVQMMYQIGLFRVASMASEKMKILELPFASGTMSMLVLLPDEVSGLEQLESIINFEKLTEWTSSNVMEERKIKVYLPRMKMEEKYNLTSVLMAMGITDVFSSSANLSGISSAESLKISQAVHAAHAEINEAGREVVGSAEAGVDAASVSEEFRADHPFLFCIKHIATNAVLFFGRCVSP

SEQ ID NO: 37 - protein, 500 aa, synthetic construct
  source 1..500: note = VAMP3-OVA
MSTGPTAATGSNRRLQQTQNQVDEVVDIMRVNVDKVLERDQKLSELDDRADALQAGASQFETSAAKLKRKYWWKNCKMWAIGITVLVIFIIIIIVWVVSSGGGGSGGGGSGGGGSGSIGAASMEFCFDVFKELKVHHANENIFYCPIAIMSALAMVYLGAKDSTRTQINKVVRFDKLPGFGDSIEAQCGTSVNVHSSLRDILNQITKPNDVYSFSLASRLYAEERYPILPEYLQCVKELYRGGLEPINFQTAADQARELINSWVESQTNGIIRNVLQPSSVDSQTAMVLVNAIVFKGLWEKTFKDEDTQAMPFRVTEQESKPVQMMYQIGLFRVASMASEKMKILELPFASGTMSMLVLLPDEVSGLEQLESIINFEKLTEWTSSNVMEERKIKVYLPRMKMEEKYNLTSVLMAMGITDVFSSSANLSGISSAESLKISQAVHAAHAEINEAGREVVGSAEAGVDAASVSEEFRADHPFLFCIKHIATNAVLFFGRCVSP

SEQ ID NO: 38 - protein, 541 aa, synthetic construct
  source 1..541: note = VAMP4-OVA
MPPKFKRHLNDDDVTGSVKSERRNLLEDDSDEEEDFFLRGPSGPRFGPRNDKIKHVQNQVDEVIDVMQENITKVIERGERLDELQDKSESLSDNATAFSNRSKQLRRQMWWRGCKIKAIMALVAAILLLVIIILIVMKYRTGGGGSGGGGSGGGGSGSIGAASMEFCFDVFKELKVHHANENIFYCPIAIMSALAMVYLGAKDSTRTQINKVVRFDKLPGFGDSIEAQCGTSVNVHSSLRDILNQITKPNDVYSFSLASRLYAEERYPILPEYLQCVKELYRGGLEPINFQTAADQARELINSWVESQTNGIIRNVLQPSSVDSQTAMVLVNAIVFKGLWEKTFKDEDTQAMPFRVTEQESKPVQMMYQIGLFRVASMASEKMKILELPFASGTMSMLVLLPDEVSGLEQLESIINFEKLTEWTSSNVMEERKIKVYLPRMKMEEKYNLTSVLMAMGITDVFSSSANLSGISSAESLKISQAVHAAHAEINEAGREVVGSAEAGVDAASVSEEFRADHPFLFCIKHIATNAVLFFGRCVSP

SEQ ID NO: 39 - protein, 500 aa, synthetic construct
  source 1..500: note = VAMP8-OVA
MEEASEGGGNDRVRNLQSEVEGVKNIMTQNVERILARGENLEHLRNKTEDLEATSEHFKTTSQKVARKFWWKNVKMIVLICVIVFIIILFIVLFATGAFSGGGGSGGGGSGGGGSGSIGAASMEFCFDVFKELKVHHANENIFYCPIAIMSALAMVYLGAKDSTRTQINKVVRFDKLPGFGDSIEAQCGTSVNVHSSLRDILNQITKPNDVYSFSLASRLYAEERYPILPEYLQCVKELYRGGLEPINFQTAADQARELINSWVESQTNGIIRNVLQPSSVDSQTAMVLVNAIVFKGLWEKTFKDEDTQAMPFRVTEQESKPVQMMYQIGLFRVASMASEKMKILELPFASGTMSMLVLLPDEVSGLEQLESIINFEKLTEWTSSNVMEERKIKVYLPRMKMEEKYNLTSVLMAMGITDVFSSSANLSGISSAESLKISQAVHAAHAEINEAGREVVGSAEAGVDAASVSEEFRADHPFLFCIKHIATNAVLFFGRCVSP

SEQ ID NO: 40 - protein, 632 aa, synthetic construct
  source 1..632: note = VTI1B-OVA
MASSAASSEHFEKLHEIFRGLHEDLQGVPERLLGTAGTEEKKKLIRDFDEKQQEANETLAEMEEELRYAPLSFRNPMMSKLRNYRKDLAKLHREVRSTPLTATPGGRGDMKYGIYAVENEHMNRLQSQRAMLLQGTESLNRATQSIERSHRIATETDQIGSEIIEELGEQRDQLERTKSRLVNTSENLSKSRKILRSMSRKVTTNKLLLSIIILLELAILGGLVYYKFFRSHGGGGSGGGGSGGGGSGSIGAASMEFCFDVFKELKVHHANENIFYCPIAIMSALAMVYLGAKDSTRTQINKVVRFDKLPGFGDSIEAQCGTSVNVHSSLRDILNQITKPNDVYSFSLASRLYAEERYPILPEYLQCVKELYRGGLEPINFQTAADQARELINSWVESQTNGIIRNVLQPSSVDSQTAMVLVNAIVFKGLWEKTFKDEDTQAMPFRVTEQESKPVQMMYQIGLFRVASMASEKMKILELPFASGTMSMLVLLPDEVSGLEQLESIINFEKLTEWTSSNVMEERKIKVYLPRMKMEEKYNLTSVLMAMGITDVFSSSANLSGISSAESLKISQAVHAAHAEINEAGREVVGSAEAGVDAASVSEEFRADHPFLFCIKHIATNAVLFFGRCVSP

SEQ ID NO: 41 - protein, 650 aa, synthetic construct
  source 1..650: note = GOSR1-OVA
MAAGTSSYWEDLRKQARQLENELDLKLVSFSKLCTSYSHSSTRDGRRDRYSSDTTPLLNGSSQDRMFETMAIEIEQLLARLTGVNDKMAEYTNSAGVPSLNAALMHTLQRHRDILQDYTHEFHKTKANFMAIRERENLMGSVRKDIESYKSGSGVNNRRTELFLKEHDHLRNSDRLIEETISIAMATKENMTSQRGMLKSIHSKMNTLANRFPAVNSLIQRINLRKRRDSLILGGVIGICTILLLLYAFHGGGGSGGGGSGGGGSGSIGAASMEFCFDVFKELKVHHANENIFYCPIAIMSALAMVYLGAKDSTRTQINKVVRFDKLPGFGDSIEAQCGTSVNVHSSLRDILNQITKPNDVYSFSLASRLYAEERYPILPEYLQCVKELYRGGLEPINFQTAADQARELINSWVESQTNGIIRNVLQPSSVDSQTAMVLVNAIVFKGLWEKTFKDEDTQAMPFRVTEQESKPVQMMYQIGLFRVASMASEKMKILELPFASGTMSMLVLLPDEVSGLEQLESIINFEKLTEWTSSNVMEERKIKVYLPRMKMEEKYNLTSVLMAMGITDVFSSSANLSGISSAESLKISQAVHAAHAEINEAGREVVGSAEAGVDAASVSEEFRADHPFLFCIKHIATNAVLFFGRCVSP

SEQ ID NO: 42 - protein, 518 aa, synthetic construct
  source 1..518: note = BET1-OVA
MRRAGLGEGVPPGNYGNYGYANSGYSACEEENERLTESLRSKVTAIKSLSIEIGHEVKTQNKLLAEMDSQFDSTTGFLGKTMGKLKILSRGSQTKLLCYMMLFSLFVFFIIYWIIKLRGGGGSGGGGSGGGGSGSIGAASMEFCFDVFKELKVHHANENIFYCPIAIMSALAMVYLGAKDSTRTQINKVVRFDKLPGFGDSIEAQCGTSVNVHSSLRDILNQITKPNDVYSFSLASRLYAEERYPILPEYLQCVKELYRGGLEPINFQTAADQARELINSWVESQTNGIIRNVLQPSSVDSQTAMVLVNAIVFKGLWEKTFKDEDTQAMPFRVTEQESKPVQMMYQIGLFRVASMASEKMKILELPFASGTMSMLVLLPDEVSGLEQLESIINFEKLTEWTSSNVMEERKIKVYLPRMKMEEKYNLTSVLMAMGITDVFSSSANLSGISSAESLKISQAVHAAHAEINEAGREVVGSAEAGVDAASVSEEFRADHPFLFCIKHIATNAVLFFGRCVSP

SEQ ID NO: 43 - protein, 690 aa, synthetic construct
  source 1..690: note = BET1L-OVA
MAFCAILLVPSLCRMPSLPTSPWAFPVHWAGFMFKPLDWQGNDFFPPQDEVLAPCLGIKTPLKHEPCASLPFSVLFQSSASQSLLGTMGSLSPHLCGHTMCPVNPELPLSFQADHRSAQPDACSPLCHPSSLLPSFHTASLPFSIHAHHSPLPCDLDPPLYLAETVSLLEEWGPPSSCPMQCKLTSHPARLTHLPPCLWGFAVALKPSWAGLAPSLLPPPRMSLCRPLSFLRHQCPWLPWQAHQGLVPWSPSMVAAACIVSPSGHCRCQPFIPHVFLGHGGLTSVSGECGGGGGSGGGGSGGGGSGSIGAASMEFCFDVFKELKVHHANENIFYCPIAIMSALAMVYLGAKDSTRTQINKVVRFDKLPGFGDSIEAQCGTSVNVHSSLRDILNQITKPNDVYSFSLASRLYAEERYPILPEYLQCVKELYRGGLEPINFQTAADQARELINSWVESQTNGIIRNVLQPSSVDSQTAMVLVNAIVFKGLWEKTFKDEDTQAMPFRVTEQESKPVQMMYQIGLFRVASMASEKMKILELPFASGTMSMLVLLPDEVSGLEQLESIINFEKLTEWTSSNVMEERKIKVYLPRMKMEEKYNLTSVLMAMGITDVFSSSANLSGISSAESLKISQAVHAAHAEINEAGREVVGSAEAGVDAASVSEEFRADHPFLFCIKHIATNAVLFFGRCVSP

SEQ ID NO: 44 - protein, 615 aa, synthetic construct
  source 1..615: note = SEC22B-OVA
MVLLTMIARVADGLPLAASMQEDEQSGRDLQQYQSQAKQLFRKLNEQSPTRCTLEAGAMTFHYIIEQGVCYLVLCEAAFPKKLAFAYLEDLHSEFDEQHGKKVPTVSRPYSFIEFDTFIQKTKKLYIDSRARRNLGSINTELQDVQRIMVANIEEVLQRGEALSALDSKANNLSSLSKKYRQDAKYLNMRSTYAKLAAVAVFFIMLIVYVRFWWLGGGGSGGGGSGGGGSGSIGAASMEFCFDVFKELKVHHANENIFYCPIAIMSALAMVYLGAKDSTRTQINKVVRFDKLPGFGDSIEAQCGTSVNVHSSLRDILNQITKPNDVYSFSLASRLYAEERYPILPEYLQCVKELYRGGLEPINFQTAADQARELINSWVESQTNGIIRNVLQPSSVDSQTAMVLVNAIVFKGLWEKTFKDEDTQAMPFRVTEQESKPVQMMYQIGLFRVASMASEKMKILELPFASGTMSMLVLLPDEVSGLEQLESIINFEKLTEWTSSNVMEERKIKVYLPRMKMEEKYNLTSVLMAMGITDVFSSSANLSGISSAESLKISQAVHAAHAEINEAGREVVGSAEAGVDAASVSEEFRADHPFLFCIKHIATNAVLFFGRCVSP

SEQ ID NO: 45 - protein, 659 aa, synthetic construct
  source 1..659: note = USE1-OVA
MAASRLELNLVRLLSRCEAMAAEKRDPDEWRLEKYVGALEDMLQALKVHASKPASEVINEYSWKVDFLKGMLQAEKLTSSSEKALANQFLAPGRVPTTARERVPATKTVHLQSRARYTSEMRSELLGTDSAEPEMDVRKRTGVAGSQPVSEKQLAAELDLVLQRHQNLQEKLAEEMLGLARSLKTNTLAAQSVIKKDNQTLSHSLKMADQNLEKLKTESERLEQHTQKSVNWLLWAMLIIVCFIFISMILFIRIMPKLKGGGGSGGGGSGGGGSGSIGAASMEFCFDVFKELKVHHANENIFYCPIAIMSALAMVYLGAKDSTRTQINKVVRFDKLPGFGDSIEAQCGTSVNVHSSLRDILNQITKPNDVYSFSLASRLYAEERYPILPEYLQCVKELYRGGLEPINFQTAADQARELINSWVESQTNGIIRNVLQPSSVDSQTAMVLVNAIVFKGLWEKTFKDEDTQAMPFRVTEQESKPVQMMYQIGLFRVASMASEKMKILELPFASGTMSMLVLLPDEVSGLEQLESIINFEKLTEWTSSNVMEERKIKVYLPRMKMEEKYNLTSVLMAMGITDVFSSSANLSGISSAESLKISQAVHAAHAEINEAGREVVGSAEAGVDAASVSEEFRADHPFLFCIKHIATNAVLFFGRCVSP

SEQ ID NO: 46 - protein, 626 aa, synthetic construct
  source 1..626: note = VAMP7-pc-OVA
MAILFAVVARGTTILAKHAWCGGNFLEVTEQILAKIPSENNKLTYSHGNYLFHYICQDRIVYLCITDDDFERSRAFNFLNEIKKRFQTTYGSRAQTALPYAMNSEFSSVLAAQLKHHSENKGLDKVMETQAQVDELKGIMVRNIDLVAQRGERLELLIDKTENLVDSSVTFKTTSRNLARAMCMKNLKLTIIIIIVSIVFIYIIVSPLCGGFTWPSCVKKSGGGGSGGGGSGGGGSRRARRGSIGAASMEFCFDVFKELKVHHANENIFYCPIAIMSALAMVYLGAKDSTRTQINKVVRFDKLPGFGDSIEAQCGTSVNVHSSLRDILNQITKPNDVYSFSLASRLYAEERYPILPEYLQCVKELYRGGLEPINFQTAADQARELINSWVESQTNGIIRNVLQPSSVDSQTAMVLVNAIVFKGLWEKTFKDEDTQAMPFRVTEQESKPVQMMYQIGLFRVASMASEKMKILELPFASGTMSMLVLLPDEVSGLEQLESIINFEKLTEWTSSNVMEERKIKVYLPRMKMEEKYNLTSVLMAMGITDVFSSSANLSGISSAESLKISQAVHAAHAEINEAGREVVGSAEAGVDAASVSEEFRADHPFLFCIKHIATNAVLFFGRCVSP

SEQ ID NO: 47 - protein, 802 aa, synthetic construct
  source 1..802: note = LAMP[OVA]
MAAPGSARRPLLLLLLLLLLGLMHCASAAMFMVKNGNGTACIMANFSAAFSVNYDTKSGPKNMTFDLPSDATVVLNRSSCGKENTSDPSLVIAFGRGHTLTLNFTRNATRYSVQLMSFVYNLSDTHLFPNASSKEIKTVESITDIRADIDKKYRCVSGTQVHMNNVTVTLHDATIQAYLSNSSFSRGETRCEQDRPSPTTAPPAPPSPSPSPVPKSPSVDKYNVSGTNGTCLLASMGLQLNLTYERKDNTTVTRLLNINPNKTSASGSCGAHLVTLELHSEGTTVLLFQFGMNASSSRFFLQGIQLNTILPDARDPAFKAANGSLRALQATVGNSYKCNAEEHVRVTKAFSVNIFKVWVQAFKVEGGQFGSVEECLLDENSMGSIGAASMEFCFDVFKELKVHHANENIFYCPIAIMSALAMVYLGAKDSTRTQINKVVRFDKLPGFGDSIEAQCGTSVNVHSSLRDILNQITKPNDVYSFSLASRLYAEERYPILPEYLQCVKELYRGGLEPINFQTAADQARELINSWVESQTNGIIRNVLQPSSVDSQTAMVLVNAIVFKGLWEKTFKDEDTQAMPFRVTEQESKPVQMMYQIGLFRVASMASEKMKILELPFASGTMSMLVLLPDEVSGLEQLESIINFEKLTEWTSSNVMEERKIKVYLPRMKMEEKYNLTSVLMAMGITDVFSSSANLSGISSAESLKISQAVHAAHAEINEAGREVVGSAEAGVDAASVSEEFRADHPFLFCIKHIATNAVLFFGRCVSPLIPIAVGGALAGLVLIVLIAYLVGRKRSHAGYQTI

SEQ ID NO: 48 - DNA, 1866 bp, synthetic construct
  source 1..1866: mol_type = other DNA; note = VAMP7-OVA
atggccatcctgttcgccgtggtggctagaggcacaaccattctggccaagcacgcttggtgcggcggcaactttctggaagtgaccgagcagatcctggccaagattcccagcgagaacaacaagctgacctacagccacggcaactacctgttccactacatctgccaggaccggatcgtgtacctgtgcatcaccgacgacgacttcgagcggagcagagccttcaacttcctgaacgagatcaagaagcggttccagaccacctacggcagcagagcacaaacagccctgccttacgccatgaacagcgagttcagctctgtgctggccgctcagctgaagcaccactccgagaacaaaggcctggacaaagtgatggaaacacaggcccaggtggacgagctgaagggcatcatggtccgaaacatcgacctggtggcccagagaggcgagagactggaactgctgatcgacaagaccgagaacctggtggacagcagcgtgaccttcaagaccaccagcagaaacctggccagagccatgtgcatgaagaacctgaagctgacgatcatcatcattatcgtgtccatcgtgttcatctacatcatcgtgtccccactgtgtggcggcttcacctggcctagctgtgtgaagaaatctggcggcggaggatctggcggaggtggaagcggaggcggaggaagtggatctattggagccgccagcatggaattttgcttcgacgtgttcaaagaactgaaggtgcaccacgccaacgagaacatcttctactgccctatcgccatcatgagcgccctggctatggtgtatctgggcgccaaggacagcacccggacacagatcaacaaggtcgtcagattcgacaagctgcccggcttcggcgattctatcgaagcccagtgtggcaccagcgtgaacgtgcacagcagcctgagagacatcctgaatcagatcaccaagcctaacgacgtgtactccttcagcctggccagcagactgtacgccgaggaaagataccccatcctgcctgagtacctgcagtgcgtgaaagagctgtacagaggcggcctggaacctatcaacttccagacagccgccgaccaggccagagagctgatcaattcttgggtcgagagccagaccaacggcatcatcagaaacgtgctgcagcccagctccgtggattctcagacagccatggtgctggtcaacgccattgtgtttaaaggcctgtgggagaaaaccttcaaggacgaggacacccaggccatgcctttcagagtgacagagcaagagtccaagcctgtgcagatgatgtaccagatcggcctgtttagagtggcctccatggcctccgagaagatgaagatcctcgagctgcctttcgccagcggcaccatgtctatgctggtgctgctgcctgatgaggtgtccggactggaacagctcgagagcatcatcaacttcgagaagctgaccgagtggaccagcagcaacgtgatggaagaacggaagatcaaggtgtacctgcctcggatgaagatggaagagaagtacaacctgaccagcgtgctgatggctatgggcatcacagacgtgttctccagcagcgccaatctgagcggcatcagctctgccgagagcctgaagatttctcaggccgtgcatgctgcccacgccgagattaacgaagccggcagagaagttgtgggatctgccgaagcaggcgtggacgctgcttctgtgtctgaggaattccgggccgaccatccttttctgttctgcatcaagcacattgccaccaacgccgtgctgttctttggcagatgcgtgtccccttga

SEQ ID NO: 49 - DNA, 1974 bp, synthetic construct
  source 1..1974: mol_type = other DNA; note = GOSR2-OVA
atggatcctctgttccagcagacccacaaacaggtgcacgagatccagagctgcatgggcagactggaaaccgccgataagcagagcgtgcacatcgtggaaaatgagatccaggccagcatcgaccagatcttcagcaggctggaacggctggaaatcctgagcagcaaagagcctcctaacaagcggcagaacgcccggctgagagtggaccagctgaagtacgatgtccagcacctccagacagccctgcggaactttcagcacagaaggcacgccagagagcagcaagaacggcagagagaggaactgctgagccggaccttcaccaccaacgacagcgacaccaccattcctatggacgagagcctgcagttcaacagcagcctgcagaaagtgcacaacggcatggacgacctgatcctggacggccacaatatcctggatggcctgagaacccagcggctgacactgaagggcacccagaagaagatcctggatatcgccaacatgctgggcctgagcaacaccgtgatgcggctgattgagaagcgggccttccaggacaagtacttcatgatcgagacacggtcccaccacgtggcccagaatggacctgaactgctgtccagcagagatcctcctgccagcgcctctagatctgccggcatcatcggcatgagccaccatcctgacctgcagatccctttcgagctgagactgggcttcgagctgtggttctatcagctgctggccgtgatcagcgaccaaggcggcggaggatctggcggaggtggaagcggaggcggaggaagtggatctattggagccgccagcatggaattttgcttcgacgtgttcaaagaactgaaggtgcaccacgccaacgagaacatcttctactgccctatcgccatcatgagcgccctggctatggtgtatctgggcgccaaggacagcacccggacacagatcaacaaggtcgtcagattcgacaagctgcccggcttcggcgattctatcgaagcccagtgtggcaccagcgtgaacgtgcacagcagcctgagagacatcctgaatcagatcaccaagcctaacgacgtgtactccttcagcctggccagcagactgtacgccgaggaaagataccccatcctgcctgagtacctgcagtgcgtgaaagagctgtacagaggcggcctggaacctatcaacttccagacagccgccgaccaggccagagagctgatcaattcttgggtcgagagccagaccaacggcatcatcagaaacgtgctgcagcccagctccgtggattctcagacagccatggtgctggtcaacgccattgtgtttaaaggcctgtgggagaaaaccttcaaggacgaggacacccaggccatgcctttcagagtgacagagcaagagtccaagcctgtgcagatgatgtaccagatcggcctgtttagagtggcctccatggcctccgagaagatgaagatcctcgagctgcctttcgccagcggcaccatgtctatgctggtgctgctgcctgatgaggtgtccggactggaacagctcgagagcatcatcaacttcgagaagctgaccgagtggaccagcagcaacgtgatggaagaacggaagatcaaggtgtacctgcctcggatgaagatggaagagaagtacaacctgaccagcgtgctgatggctatgggcatcacagacgtgttctccagcagcgccaatctgagcggcatcagctctgccgagagcctgaagatttctcaggccgtgcatgctgcccacgccgagattaacgaagccggcagagaagttgtgggatctgccgaagcaggcgtggacgctgcttctgtgtctgaggaattccgggccgaccatccttttctgttctgcatcaagcacattgccaccaacgccgtgctgttctttggcagatgcgtgtccccttga

SEQ ID NO: 50 - DNA, 1950 bp, synthetic construct
  source 1..1950: mol_type = other DNA; note = STX10-OVA
atgagcctggaagatcccttctttgtcgtgcgcggcgaggtgcagaaagccgtgaatactgccagaggcctgtaccagcgttggtgcgagctgctgcaagaatctgccgctgtgggcagagaggaactggactggaccaccaacgagctgagaaacggcctgagatccatcgagtgggacctcgaggacctggaagagacaatcggcatcgtggaagccaatcctggcaagttcaaactgcctgccggcgacctgcaagagcggaaggtgttcgtggaacggatgcgggaagccgtgcaagagatgaaggaccacatggtgtctccaaccgccgtggccttcctggaacggaacaacagagagatcctggccggaaagcctgccgctcagaagtctcctagcgatctgctggatgcctctgccgtgtctgccacaagccggtacattgaggaacagcaggccacacagcagctgatcatggacgagcaggaccagcagctggaaatggtgtctggcagcatccaggtgctgaagcacatgagcggaagagtgggcgaagaactggatgagcagggcatcatgctggacgccttcgctcaagagatggatcacacccagagccggatggacggcgtgctgagaaagctggccaaagtgtcccacatgaccagcgaccgtagacagtggtgcgccattgctgtgcttgtgggagtgctgctgctggtgctgatcctgctgtttagccttggcggcggaggatctggcggaggtggaagcggaggcggaggaagtggatctattggagccgccagcatggaattttgcttcgacgtgttcaaagaactgaaggtgcaccacgccaacgagaacatcttctactgccctatcgccatcatgagcgccctggctatggtgtatctgggcgccaaggacagcacccggacacagatcaacaaggtcgtcagattcgacaagctgcccggcttcggcgattctatcgaagcccagtgtggcaccagcgtgaacgtgcacagcagcctgagagacatcctgaatcagatcaccaagcctaacgacgtgtactccttcagcctggccagcagactgtacgccgaggaaagataccccatcctgcctgagtacctgcagtgcgtgaaagagctgtacagaggcggcctggaacctatcaacttccagacagccgccgaccaggccagagagctgatcaattcttgggtcgagagccagaccaacggcatcatcagaaacgtgctgcagcccagctccgtggattctcagacagccatggtgctggtcaacgccattgtgtttaaaggcctgtgggagaaaaccttcaaggacgaggacacccaggccatgcctttcagagtgacagagcaagagtccaagcctgtgcagatgatgtaccagatcggcctgtttagagtggcctccatggcctccgagaagatgaagatcctcgagctgcctttcgccagcggcaccatgtctatgctggtgctgctgcctgatgaggtgtccggactggaacagctcgagagcatcatcaacttcgagaagctgaccgagtggaccagcagcaacgtgatggaagaacggaagatcaaggtgtacctgcctcggatgaagatggaagagaagtacaacctgaccagcgtgctgatggctatgggcatcacagacgtgttctccagcagcgccaatctgagcggcatcagctctgccgagagcctgaagatttctcaggccgtgcatgctgcccacgccgagattaacgaagccggcagagaagttgtgggatctgccgaagcaggcgtggacgctgcttctgtgtctgaggaattccgggccgaccatccttttctgttctgcatcaagcacattgccaccaacgccgtgctgttctttggcagatgcgtgtccccttga

SEQ ID NO: 51 - DNA, 2208 bp, synthetic construct
  source 1..2208: mol_type = other DNA; note = STX18-OVA
atggccgtggatatcaccctgctgtttcgggccagcgtgaaaacagtgaaaacccggaacaaggccctgggcgttgcagttggaggcggagttgatggcagcagggatgagctgttcagaagaagccccagacctaagggcgacttcagcagcagagcccgggaagtgatcagccacatcggcaagctgagagacttcctgctggaacaccggaaggactacatcaacgcctacagccacaccatgagcgagtacggcagaatgaccgacaccgagagggaccagatcgaccaggatgcccagatcttcatgcggacctgtagcgaggccatccagcagctgagaacagaggcccacaaagagatccacagccagcaagtgaaagaacacagaaccgccgtgctggacttcatcgaggactacctgaagagagtgtgcaagctgtactccgagcagcgggccatcagagtgaaaagagtggtggacaagaagcggctgagcaagctggaacccgagcctaacaccaagaccagagagagcaccagctccgagaaagtgtctcagagccccagcaaggacagcgaggaaaatcctgccaccgaggaacggcccgagaagattctggctgagacacagcctgaactcggcacctggggagatggcaagggcgaagatgaactgagccccgaagagattcagatgttcgagcaagagaaccagcggctgatcggcgagatgaacagcctgtttgacgaagtgcggcagatcgagggccgcgtggtggaaatctctcggctgcaagagatcttcaccgagaaggtcctgcagcaagaggccgagatcgacagcatccatcagctggttgtgggcgccaccgagaacatcaaagagggcaacgaggacatcagagaggccatcaagaacaacgccggcttcagagtgtggatcctgttcttcctggtcatgtgcagcttcagcctgctgttcctggattggtacgactctggcggcggaggatctggcggaggtggaagcggaggcggaggaagtggatctattggagccgccagcatggaattttgcttcgacgtgttcaaagaactgaaggtgcaccacgccaacgagaacatcttctactgccctatcgccatcatgagcgccctggctatggtgtatctgggcgccaaggacagcacccggacacagatcaacaaggtcgtcagattcgacaagctgcccggcttcggcgattctatcgaagcccagtgtggcaccagcgtgaacgtgcacagcagcctgagagacatcctgaatcagatcaccaagcctaacgacgtgtactccttcagcctggccagcagactgtacgccgaggaaagataccccatcctgcctgagtacctgcagtgcgtgaaagagctgtacagaggcggcctggaacctatcaacttccagacagccgccgaccaggccagagagctgatcaattcttgggtcgagagccagaccaacggcatcatcagaaacgtgctgcagcccagctccgtggattctcagacagccatggtgctggtcaacgccattgtgtttaaaggcctgtgggagaaaaccttcaaggacgaggacacccaggccatgcctttcagagtgacagagcaagagtccaagcctgtgcagatgatgtaccagatcggcctgtttagagtggcctccatggcctccgagaagatgaagatcctcgagctgcctttcgccagcggcaccatgtctatgctggtgctgctgcctgatgaggtgtccggactggaacagctcgagagcatcatcaacttcgagaagctgaccgagtggaccagcagcaacgtgatggaagaacggaagatcaaggtgtacctgcctcggatgaagatggaagagaagtacaacctgaccagcgtgctgatggctatgggcatcacagacgtgttctccagcagcgccaatctgagcggcatcagctctgccgagagcctgaagatttctcaggccgtgcatgctgcccacgccgagattaacgaagccggcagagaagttgtgggatctgccgaagcaggcgtggacgctgcttctgtgtctgaggaattccgggccgaccatccttttctgttctgcatcaagcacattgccaccaacgccgtgctgttctttggcagatgcgtgtccccttga

SEQ ID NO: 52 - DNA, 2016 bp, synthetic construct
  source 1..2016: mol_type = other DNA; note = BNIP1-OVA
atggctgctcctcaggatgtgcacgtgcggatctgcaatcaagagatcgtgaagttcgacctggaagtgaaggccctgatccaggacatcagagactgtagcggacctctgagcgccctgaccgagctgaacaccaaagtgaaagagaagttccagcagctgcggcaccggatccagcctgtgctgtatcagagagccttcatctggaccgccagcaccttctttttcaaactgacctacagcctgaccgacttcagcagcacccagcacgacttcaacagccctaccacacctgtgaccttcagcgatctggaacagctggccaaagagcaggacaaagagagcgagaaacagctgctgctgcaagaggtggaaaaccacaaaaagcagatgctgagcaaccaggcctcctggcggaaggccaatctgacatgcaagatcgccatcgacaacctggaaaaggccgagctgctccaaggcggcgatctgctgagacagagaaagaccaccaaagagtctctggcccagaccagctccaccatcaccgaatctctgatgggcatcagcagaatgatggcccagcaggtccagcagagcgaggaagccatgcagagcctggtcaccagcagcagaacaatcctggacgccaacgaggaattcaagagcatgagcggcaccatccagctgggcagaaagctgatcaccaagtacaacagaagagagctgaccgacaagctgctgatcttcctggctctggccctgtttctggccaccgtgctgtacatcgtgaagaagcggctgttcccattccttggcggcggaggatctggcggaggtggaagcggaggcggaggaagtggatctattggagccgccagcatggaattttgcttcgacgtgttcaaagaactgaaggtgcaccacgccaacgagaacatcttctactgccctatcgccatcatgagcgccctggctatggtgtatctgggcgccaaggacagcacccggacacagatcaacaaggtcgtcagattcgacaagctgcccggcttcggcgattctatcgaagcccagtgtggcaccagcgtgaacgtgcacagcagcctgagagacatcctgaatcagatcaccaagcctaacgacgtgtactccttcagcctggccagcagactgtacgccgaggaaagataccccatcctgcctgagtacctgcagtgcgtgaaagagctgtacagaggcggcctggaacctatcaacttccagacagccgccgaccaggccagagagctgatcaattcttgggtcgagagccagaccaacggcatcatcagaaacgtgctgcagcccagctccgtggattctcagacagccatggtgctggtcaacgccattgtgtttaaaggcctgtgggagaaaaccttcaaggacgaggacacccaggccatgcctttcagagtgacagagcaagagtccaagcctgtgcagatgatgtaccagatcggcctgtttagagtggcctccatggcctccgagaagatgaagatcctcgagctgcctttcgccagcggcaccatgtctatgctggtgctgctgcctgatgaggtgtccggactggaacagctcgagagcatcatcaacttcgagaagctgaccgagtggaccagcagcaacgtgatggaagaacggaagatcaaggtgtacctgcctcggatgaagatggaagagaagtacaacctgaccagcgtgctgatggctatgggcatcacagacgtgttctccagcagcgccaatctgagcggcatcagctctgccgagagcctgaagatttctcaggccgtgcatgctgcccacgccgagattaacgaagccggcagagaagttgtgggatctgccgaagcaggcgtggacgctgcttctgtgtctgaggaattccgggccgaccatccttttctgttctgcatcaagcacattgccaccaacgccgtgctgttctttggcagatgcgtgtccccttga

SEQ ID NO: 53 - DNA, 1986 bp, synthetic construct
  source 1..1986: mol_type = other DNA; note = STX7-OVA
atgagctacacacctggcgttggcggagatcctgctcagctggcccagagaatcagcagcaacatccagaaaatcacccagtgcagcgtggaaatccagcggaccctgaatcagctgggcacccctcaggatagccctgagctgagacagcagctgcagcagaagcagcagtacaccaaccagctggccaaagagacagacaagtacatcaaagagttcggcagcctgcctaccacacctagcgagcagagacagcggaagatccagaaagacagactggtggccgagttcaccaccagcctgaccaacttccagaaggtgcagaggcaggccgctgagcgcgagaaagaatttgtggccagagtgcgggccagcagcagagtgtcaggatcctttccagaggacagctccaaagagcggaacctggtttcctgggagagccagacacagcctcaggtgcaggtccaggacgaggaaatcaccgaggacgacctgagactgatccacgagagagagtccagcatccggcagctggaagccgacatcatggacatcaacgagatcttcaaggacctgggcatgatgattcacgagcagggcgacgtgatcgacagcatcgaggccaacgtggaaaacgccgaagtgcatgtgcagcaggccaaccagcagctgtctagagccgccgactaccagcgcaagagcagaaagaccctgtgcatcatcatcctgatcctggtcatcggcgtggccatcatctccctgatcatctggggcctgaaccatggcggcggaggatctggcggaggtggaagcggaggcggaggaagtggatctattggagccgccagcatggaattttgcttcgacgtgttcaaagaactgaaggtgcaccacgccaacgagaacatcttctactgccctatcgccatcatgagcgccctggctatggtgtatctgggcgccaaggacagcacccggacacagatcaacaaggtcgtcagattcgacaagctgcccggcttcggcgattctatcgaagcccagtgtggcaccagcgtgaacgtgcacagcagcctgagagacatcctgaatcagatcaccaagcctaacgacgtgtactccttcagcctggccagcagactgtacgccgaggaaagataccccatcctgcctgagtacctgcagtgcgtgaaagagctgtacagaggcggcctggaacctatcaacttccagacagccgccgaccaggccagagagctgatcaattcttgggtcgagagccagaccaacggcatcatcagaaacgtgctgcagcccagctccgtggattctcagacagccatggtgctggtcaacgccattgtgtttaaaggcctgtgggagaaaaccttcaaggacgaggacacccaggccatgcctttcagagtgacagagcaagagtccaagcctgtgcagatgatgtaccagatcggcctgtttagagtggcctccatggcctccgagaagatgaagatcctcgagctgcctttcgccagcggcaccatgtctatgctggtgctgctgcctgatgaggtgtccggactggaacagctcgagagcatcatcaacttcgagaagctgaccgagtggaccagcagcaacgtgatggaagaacggaagatcaaggtgtacctgcctcggatgaagatggaagagaagtacaacctgaccagcgtgctgatggctatgggcatcacagacgtgttctccagcagcgccaatctgagcggcatcagctctgccgagagcctgaagatttctcaggccgtgcatgctgcccacgccgagattaacgaagccggcagagaagttgtgggatctgccgaagcaggcgtggacgctgcttctgtgtctgaggaattccgggccgaccatccttttctgttctgcatcaagcacattgccaccaacgccgtgctgttctttggcagatgcgtgtccccttga

SEQ ID NO: 54 - DNA, 1875 bp, synthetic construct
  source 1..1875: mol_type = other DNA; note = VTI1A-OVA
atgagcagcgacttcgagggctacgagcaggattttgccgtgctgaccgccgagatcaccagcaagattgccagagtgcccagactgcctcctgacgagaagaaacagatggtggccaacgtggaaaagcagctggaagaggccaaagaactgctggaacagatggacctggaagtgcgcgagatccctccacagagcagaggcatgtacagcaaccggatgcggagctacaagcaagagatgggcaagctggaaaccgacttcaagcggagcagaatcgcctacagcgacgaagtgcggaatgagctgctgggcgacgatggcaacagcagcgagaaccagctgatcaagctgcgggaagagagagcccatctgctggacaacaccgagcggctggaaagaagcagcagaaggctggaagccggctatcagatcgccgtggaaactgagcagatcggccaagagatgctggaaaacctgagccacgacagagagaagatccagcgggccagagagcggctgagagagacagacgccaatctgggcaagagcagcaggattctgaccggcatgctgcggcggatcatccagaataggatcctgctggtcatcctgggcatcatcgtggtcatcaccatcctgatggccattaccttcagcgtgcggcggcatggcggcggaggatctggcggaggtggaagcggaggcggaggaagtggatctattggagccgccagcatggaattttgcttcgacgtgttcaaagaactgaaggtgcaccacgccaacgagaacatcttctactgccctatcgccatcatgagcgccctggctatggtgtatctgggcgccaaggacagcacccggacacagatcaacaaggtcgtcagattcgacaagctgcccggcttcggcgattctatcgaagcccagtgtggcaccagcgtgaacgtgcacagcagcctgagagacatcctgaatcagatcaccaagcctaacgacgtgtactccttcagcctggccagcagactgtacgccgaggaaagataccccatcctgcctgagtacctgcagtgcgtgaaagagctgtacagaggcggcctggaacctatcaacttccagacagccgccgaccaggccagagagctgatcaattcttgggtcgagagccagaccaacggcatcatcagaaacgtgctgcagcccagctccgtggattctcagacagccatggtgctggtcaacgccattgtgtttaaaggcctgtgggagaaaaccttcaaggacgaggacacccaggccatgcctttcagagtgacagagcaagagtccaagcctgtgcagatgatgtaccagatcggcctgtttagagtggcctccatggcctccgagaagatgaagatcctcgagctgcctttcgccagcggcaccatgtctatgctggtgctgctgcctgatgaggtgtccggactggaacagctcgagagcatcatcaacttcgagaagctgaccgagtggaccagcagcaacgtgatggaagaacggaagatcaaggtgtacctgcctcggatgaagatggaagagaagtacaacctgaccagcgtgctgatggctatgggcatcacagacgtgttctccagcagcgccaatctgagcggcatcagctctgccgagagcctgaagatttctcaggccgtgcatgctgcccacgccgagattaacgaagccggcagagaagttgtgggatctgccgaagcaggcgtggacgctgcttctgtgtctgaggaattccgggccgaccatccttttctgttctgcatcaagcacattgccaccaacgccgtgctgttctttggcagatgcgtgtccccttga

SEQ ID NO: 55 - DNA, 2178 bp, synthetic construct
  source 1..2178: mol_type = other DNA; note = STX16-OVA
atggccaccagaaggctgacagacgctttcctgctgctgcggaacaacagcatccagaacagacagctgctggccgaacaggtgtccagccacatcacatctagccctctgcacagcagatctatcgccgccgagctggatgagctggccgatgatagaatggccctggtgtccggcatctctctggatcctgaagccgccatcggcgtgaccaaacggcctcctcctaaatgggttgacggcgtggacgagatccagtacgacgtgggcagaatcaagcagaagatgaaggaactggccagcctgcacgacaagcacctgaacagacccacactggacgacagcagcgaggaagaacacgccatcgagatcaccacacaagagatcacccagctgttccaccggtgccagagagctgttcaggccctgccttctagagccagagcctgctctgagcaagagggcagactgctgggaaacgtggtggcttctctggctcaggctctgcaagagctgagcaccagctttagacacgcccagagcggctacctgaagcggatgaagaaccgggaagagagatcccagcacttcttcgacaccagcgtgcccctgatggacgacggcgacgataataccctgtaccacagaggcttcaccgaggaccagctcgtgctggttgagcagaacaccctgatggtggaagaacgcgagcgcgagatcagacagatcgtgcagagcatcagcgacctgaacgagatcttcagagatctgggcgccatgatcgtggaacagggcaccgtgctggaccggatcgactacaatgtggaacagagctgcatcaagaccgaggacggactgaagcagctgcacaaagccgagcagtaccagaaaaagaatcggaagatgctggtcatcctgatcctgttcgtgatcatcatcgtgctgatcgtggtgctcgtgggcgtgaagtctagaggcggcggaggatctggcggaggtggaagcggaggcggaggaagtggatctattggagccgccagcatggaattttgcttcgacgtgttcaaagaactgaaggtgcaccacgccaacgagaacatcttctactgccctatcgccatcatgagcgccctggctatggtgtatctgggcgccaaggacagcacccggacacagatcaacaaggtcgtcagattcgacaagctgcccggcttcggcgattctatcgaagcccagtgtggcaccagcgtgaacgtgcacagcagcctgagagacatcctgaatcagatcaccaagcctaacgacgtgtactccttcagcctggccagcagactgtacgccgaggaaagataccccatcctgcctgagtacctgcagtgcgtgaaagagctgtacagaggcggcctggaacctatcaacttccagacagccgccgaccaggccagagagctgatcaattcttgggtcgagagccagaccaacggcatcatcagaaacgtgctgcagcccagctccgtggattctcagacagccatggtgctggtcaacgccattgtgtttaaaggcctgtgggagaaaaccttcaaggacgaggacacccaggccatgcctttcagagtgacagagcaagagtccaagcctgtgcagatgatgtaccagatcggcctgtttagagtggcctccatggcctccgagaagatgaagatcctcgagctgcctttcgccagcggcaccatgtctatgctggtgctgctgcctgatgaggtgtccggactggaacagctcgagagcatcatcaacttcgagaagctgaccgagtggaccagcagcaacgtgatggaagaacggaagatcaaggtgtacctgcctcggatgaagatggaagagaagtacaacctgaccagcgtgctgatggctatgggcatcacagacgtgttctccagcagcgccaatctgagcggcatcagctctgccgagagcctgaagatttctcaggccgtgcatgctgcccacgccgagattaacgaagccggcagagaagttgtgggatctgccgaagcaggcgtggacgctgcttctgtgtctgaggaattccgggccgaccatccttttctgttctgcatcaagcacattgccaccaacgccgtgctgttctttggcagatgcgtgtccccttga

SEQ ID NO: 56 - DNA, 2268 bp, synthetic construct
  source 1..2268: mol_type = other DNA; note = STX5-OVA
atgattccccggaagagatacggcagcaagaacaccgatcagggcgtgtacctgggcctgagcaaaacacaggtgctgtctccagccacagccggcagctctagctctgatattgctcccctgcctcctcctgtgacactggttcctccaccacctgacaccatgagctgcagagacagaacccaagagttcctgagcgcctgcaagagcctgcagaccagacagaatggcatccagaccaacaagcccgctctgagagccgtgcggcagagaagcgagtttaccctgatggccaagcggatcggcaaggacctgagcaacaccttcgccaagctggaaaagctgaccatcctggccaagagaaagagcctgttcgacgacaaggccgtggaaatcgaggaactgacctacatcatcaagcaggacatcaacagcctgaacaagcagatcgcccagctgcaggacttcgtcagagccaagggaagccagagcggcagacacctccagacacacagcaacaccatcgtggtgtccctgcagagcaagctggcctccatgagcaacgacttcaagagcgtgctggaagtgcggaccgagaacctgaagcagcagcggtctagaagagagcagttcagcagagcccctgtgtctgctctgcccctggctcctaatcatcttggaggcggagctgtggtgctgggagccgaatctcacgcctctaaggacgtggccatcgacatgatggacagcagaaccagccagcagctgcaactgatcgacgagcaggacagctacatccagagcagagccgacaccatgcagaacatcgagagcacaatcgtggaactgggcagcatctttcagcagctggcccacatggtcaaagagcaagaggaaaccatccagcgcatcgacgagaatgtgctgggcgctcagctggatgtggaagccgctcactctgagatcctgaagtactttcagagcgtgaccagcaaccggtggctgatggtcaagatcttcctgatcctgatcgtgttctttattatcttcgtcgtgttcctggctggcggcggaggatctggcggaggtggaagcggaggcggaggaagtggatctattggagccgccagcatggaattttgcttcgacgtgttcaaagaactgaaggtgcaccacgccaacgagaacatcttctactgccctatcgccatcatgagcgccctggctatggtgtatctgggcgccaaggacagcacccggacacagatcaacaaggtcgtcagattcgacaagctgcccggcttcggcgattctatcgaagcccagtgtggcaccagcgtgaacgtgcacagcagcctgagagacatcctgaatcagatcaccaagcctaacgacgtgtactccttcagcctggccagcagactgtacgccgaggaaagataccccatcctgcctgagtacctgcagtgcgtgaaagagctgtacagaggcggcctggaacctatcaacttccagacagccgccgaccaggccagagagctgatcaattcttgggtcgagagccagaccaacggcatcatcagaaacgtgctgcagcccagctccgtggattctcagacagccatggtgctggtcaacgccattgtgtttaaaggcctgtgggagaaaaccttcaaggacgaggacacccaggccatgcctttcagagtgacagagcaagagtccaagcctgtgcagatgatgtaccagatcggcctgtttagagtggcctccatggcctccgagaagatgaagatcctcgagctgcctttcgccagcggcaccatgtctatgctggtgctgctgcctgatgaggtgtccggactggaacagctcgagagcatcatcaacttcgagaagctgaccgagtggaccagcagcaacgtgatggaagaacggaagatcaaggtgtacctgcctcggatgaagatggaagagaagtacaacctgaccagcgtgctgatggctatgggcatcacagacgtgttctccagcagcgccaatctgagcggcatcagctctgccgagagcctgaagatttctcaggccgtgcatgctgcccacgccgagattaacgaagccggcagagaagttgtgggatctgccgaagcaggcgtggacgctgcttctgtgtctgaggaattccgggccgaccatccttttctgttctgcatcaagcacattgccaccaacgccgtgctgttctttggcagatgcgtgtccccttga

SEQ ID NO: 57 - DNA, 1968 bp, synthetic construct
  source 1..1968: mol_type = other DNA; note = STX6-OVA
atgagcatggaagatccattcttcgtggtcaagggcgaagtgcagaaagccgtgaacacagcccagggcctgttccagagatggacagagctgctgcaggaccctagcaccgccaccagagaggaaatcgactggaccaccaacgagctgcggaacaacctgagatccatcgagtgggacctcgaggacctggacgagacaatcagcatcgtggaagccaatcctcggaagttcaacctggacgccaccgagctgagcatcagaaaggccttcatcaccagcaccagacaggtcgtgcgggacatgaaggaccagatgagcacaagctctgtgcaggctctggccgagcggaagaatagacaggctctgctgggcgatagcggcagccagaattggagcaccggcaccacagataagtacggcagactggatagagagctgcagcgggccaacagccacttcatcgaagaacagcaggcccagcagcagctgatcgtcgagcagcaggatgagcagctggaactggtgtctggctctatcggcgtgctgaagaacatgagccagagaatcggcggcgaactggaagaacaggccgtgatgctggaagatttcagccacgagctggaaagcacccagagcaggctggacaacgtgatgaagaagctggccaaggtttcccacatgaccagcgaccgtagacagtggtgcgccattgccatcctgtttgccgtgctgctggtggtgctgatcctgttcctggtgcttggcggcggaggatctggcggaggtggaagcggaggcggaggaagtggatctattggagccgccagcatggaattttgcttcgacgtgttcaaagaactgaaggtgcaccacgccaacgagaacatcttctactgccctatcgccatcatgagcgccctggctatggtgtatctgggcgccaaggacagcacccggacacagatcaacaaggtcgtcagattcgacaagctgcccggcttcggcgattctatcgaagcccagtgtggcaccagcgtgaacgtgcacagcagcctgagagacatcctgaatcagatcaccaagcctaacgacgtgtactccttcagcctggccagcagactgtacgccgaggaaagataccccatcctgcctgagtacctgcagtgcgtgaaagagctgtacagaggcggcctggaacctatcaacttccagacagccgccgaccaggccagagagctgatcaattcttgggtcgagagccagaccaacggcatcatcagaaacgtgctgcagcccagctccgtggattctcagacagccatggtgctggtcaacgccattgtgtttaaaggcctgtgggagaaaaccttcaaggacgaggacacccaggccatgcctttcagagtgacagagcaagagtccaagcctgtgcagatgatgtaccagatcggcctgtttagagtggcctccatggcctccgagaagatgaagatcctcgagctgcctttcgccagcggcaccatgtctatgctggtgctgctgcctgatgaggtgtccggactggaacagctcgagagcatcatcaacttcgagaagctgaccgagtggaccagcagcaacgtgatggaagaacggaagatcaaggtgtacctgcctcggatgaagatggaagagaagtacaacctgaccagcgtgctgatggctatgggcatcacagacgtgttctccagcagcgccaatctgagcggcatcagctctgccgagagcctgaagatttctcaggccgtgcatgctgcccacgccgagattaacgaagccggcagagaagttgtgggatctgccgaagcaggcgtggacgctgcttctgtgtctgaggaattccgggccgaccatccttttctgttctgcatcaagcacattgccaccaacgccgtgctgttctttggcagatgcgtgtccccttga

SEQ ID NO: 58 - DNA, 1911 bp, synthetic construct
  source 1..1911: mol_type = other DNA; note = STX8-OVA
atggctcccgatccatggttcagcacctacgacagcacctgtcagatcgcccaagagatcgccgagaagatccagcagcggaaccagtacgagcggaagggcgagaaagcccctaagctgaccgtgaccattagagccctgctgcagaacctgaaagagaagatcgccctgctgaaggatctgctgctgagagccgtgtctacccaccagatcacacagctggaaggcgaccgcagacagaacctgctggatgacctggtcaccagagagagactgctgctggcctccttcaagaacgaaggcgccgagcctgacctgatcagatccagcctgatgagcgaggaagccaagagaggcgcccctaatccttggctgttcgaggaacccgaggaaaccagaggcctgggcttcgacgagatcagacagcagcagcaaaagatcatccaagagcaggacgccggcctggatgccctgtctagcatcatcagccggcagaaacagatgggccaagagattggcaacgagctggacgagcagaacgagatcatcgacgacctggccaacctggtggaaaacaccgacgagaagctgcggaacgagactcggagagtgaacatggtggaccggaagtctgccagctgcgggatgatcatggttatcctgttgctgctggtggccatcgtggtggtggctgtgtggcctacaaatggcggcggaggatctggcggaggtggaagcggaggcggaggaagtggatctattggagccgccagcatggaattttgcttcgacgtgttcaaagaactgaaggtgcaccacgccaacgagaacatcttctactgccctatcgccatcatgagcgccctggctatggtgtatctgggcgccaaggacagcacccggacacagatcaacaaggtcgtcagattcgacaagctgcccggcttcggcgattctatcgaagcccagtgtggcaccagcgtgaacgtgcacagcagcctgagagacatcctgaatcagatcaccaagcctaacgacgtgtactccttcagcctggccagcagactgtacgccgaggaaagataccccatcctgcctgagtacctgcagtgcgtgaaagagctgtacagaggcggcctggaacctatcaacttccagacagccgccgaccaggccagagagctgatcaattcttgggtcgagagccagaccaacggcatcatcagaaacgtgctgcagcccagctccgtggattctcagacagccatggtgctggtcaacgccattgtgtttaaaggcctgtgggagaaaaccttcaaggacgaggacacccaggccatgcctttcagagtgacagagcaagagtccaagcctgtgcagatgatgtaccagatcggcctgtttagagtggcctccatggcctccgagaagatgaagatcctcgagctgcctttcgccagcggcaccatgtctatgctggtgctgctgcctgatgaggtgtccggactggaacagctcgagagcatcatcaacttcgagaagctgaccgagtggaccagcagcaacgtgatggaagaacggaagatcaaggtgtacctgcctcggatgaagatggaagagaagtacaacctgaccagcgtgctgatggctatgggcatcacagacgtgttctccagcagcgccaatctgagcggcatcagctctgccgagagcctgaagatttctcaggccgtgcatgctgcccacgccgagattaacgaagccggcagagaagttgtgggatctgccgaagcaggcgtggacgctgcttctgtgtctgaggaattccgggccgaccatccttttctgttctgcatcaagcacattgccaccaacgccgtgctgttctttggcagatgcgtgtccccttga

SEQ ID NO: 59 - DNA, 2031 bp, synthetic construct
  source 1..2031: mol_type = other DNA; note = STX12-OVA
atgagctacggccctctggacatgtacagaaaccccggaccttctggcccacagctgagagacttcagcagcatcatccagacctgcagcggcaacatccagagaatcagccaggccaccgctcagatcaagaacctgatgagccagctgggcaccaagcaggacagcagcaagctgcaagagaacctgcagcagctccagcacagcaccaaccagctggccaaagagacaaacgagctgctgaaagagctgggcagcctgcctctgcctctgagcacatctgaacagcggcagcagcggctgcagaaagaacggctgatgaacgacttcagcgccgctctgaacaacttccaggccgtgcagagaagagtgtccgagaaagagaaagagtctatcgccagagccagagccggcagcagactgtctgccgaggaaagacagcgggaagaacagctggtgtccttcgacagccacgaggaatggaaccagatgcagagccaagaggacgaggtggccatcaccgagcaggacctggaactgatcaaagagagagagacagccatccggcagctggaagccgacatcctggatgtgaaccagatcttcaaggacctggccatgatgatccacgaccagggcgacctgatcgacagcatcgaggccaatgtggaaagcagcgaggtgcacgtggaacgggctacagaacaactgcagagagccgcctactaccagaagaaaagccggaagaaaatgtgcatcctggtgctggtcctgagcgtgatcatcctgatcctgggcctgatcatctggctggtgtacaagaccaaaggcggcggaggatctggcggaggtggaagcggaggcggaggaagtggatctattggagccgccagcatggaattttgcttcgacgtgttcaaagaactgaaggtgcaccacgccaacgagaacatcttctactgccctatcgccatcatgagcgccctggctatggtgtatctgggcgccaaggacagcacccggacacagatcaacaaggtcgtcagattcgacaagctgcccggcttcggcgattctatcgaagcccagtgtggcaccagcgtgaacgtgcacagcagcctgagagacatcctgaatcagatcaccaagcctaacgacgtgtactccttcagcctggccagcagactgtacgccgaggaaagataccccatcctgcctgagtacctgcagtgcgtgaaagagctgtacagaggcggcctggaacctatcaacttccagacagccgccgaccaggccagagagctgatcaattcttgggtcgagagccagaccaacggcatcatcagaaacgtgctgcagcccagctccgtggattctcagacagccatggtgctggtcaacgccattgtgtttaaaggcctgtgggagaaaaccttcaaggacgaggacacccaggccatgcctttcagagtgacagagcaagagtccaagcctgtgcagatgatgtaccagatcggcctgtttagagtggcctccatggcctccgagaagatgaagatcctcgagctgcctttcgccagcggcaccatgtctatgctggtgctgctgcctgatgaggtgtccggactggaacagctcgagagcatcatcaacttcgagaagctgaccgagtggaccagcagcaacgtgatggaagaacggaagatcaaggtgtacctgcctcggatgaagatggaagagaagtacaacctgaccagcgtgctgatggctatgggcatcacagacgtgttctccagcagcgccaatctgagcggcatcagctctgccgagagcctgaagatttctcaggccgtgcatgctgcccacgccgagattaacgaagccggcagagaagttgtgggatctgccgaagcaggcgtggacgctgcttctgtgtctgaggaattccgggccgaccatccttttctgttctgcatcaagcacattgccaccaacgccgtgctgttctttggcagatgcgtgtccccttga

SEQ ID NO: 60 - DNA, 1503 bp, synthetic construct
  source 1..1503: mol_type = other DNA; note = VAMP3-OVA
atgagcacaggacctacagccgccacaggcagcaatagaaggctgcagcagacccagaaccaggtggacgaggtggtggacatcatgagagtgaacgtggacaaggtgctggaacgggaccagaagctgagcgagctggacgatagagccgatgctctgcaagctggcgcctctcagtttgagacatctgccgccaagctgaagcggaagtactggtggaagaactgcaagatgtgggccatcggcatcaccgtgctggtcatctttatcatcatcattatcgtgtgggtcgtgtcctctggcggcggaggatctggcggaggtggaagcggaggcggaggaagtggatctattggagccgccagcatggaattttgcttcgacgtgttcaaagaactgaaggtgcaccacgccaacgagaacatcttctactgccctatcgccatcatgagcgccctggctatggtgtatctgggcgccaaggacagcacccggacacagatcaacaaggtcgtcagattcgacaagctgcccggcttcggcgattctatcgaagcccagtgtggcaccagcgtgaacgtgcacagcagcctgagagacatcctgaatcagatcaccaagcctaacgacgtgtactccttcagcctggccagcagactgtacgccgaggaaagataccccatcctgcctgagtacctgcagtgcgtgaaagagctgtacagaggcggcctggaacctatcaacttccagacagccgccgaccaggccagagagctgatcaattcttgggtcgagagccagaccaacggcatcatcagaaacgtgctgcagcccagctccgtggattctcagacagccatggtgctggtcaacgccattgtgtttaaaggcctgtgggagaaaaccttcaaggacgaggacacccaggccatgcctttcagagtgacagagcaagagtccaagcctgtgcagatgatgtaccagatcggcctgtttagagtggcctccatggcctccgagaagatgaagatcctcgagctgcctttcgccagcggcaccatgtctatgctggtgctgctgcctgatgaggtgtccggactggaacagctcgagagcatcatcaacttcgagaagctgaccgagtggaccagcagcaacgtgatggaagaacggaagatcaaggtgtacctgcctcggatgaagatggaagagaagtacaacctgaccagcgtgctgatggctatgggcatcacagacgtgttctccagcagcgccaatctgagcggcatcagctctgccgagagcctgaagatttctcaggccgtgcatgctgcccacgccgagattaacgaagccggcagagaagttgtgggatctgccgaagcaggcgtggacgctgcttctgtgtctgaggaattccgggccgaccatccttttctgttctgcatcaagcacattgccaccaacgccgtgctgttctttggcagatgcgtgtccccttga

SEQ ID NO: 61 - DNA, 1626 bp, synthetic construct
  source 1..1626: mol_type = other DNA; note = VAMP4-OVA
atgcctccaaagttcaagcggcacctgaacgacgacgatgtgaccggctctgtgaagtccgagcggagaaacctgctggaagatgacagcgacgaggaagaggacttcttcctgcggggaccttctggccctagattcggccccagaaacgacaagatcaagcacgtgcagaaccaggtggacgaagtgatcgacgtgatgcaagagaacatcaccaaagtcatcgagcggggcgagagactggacgagctgcaggataagagcgagagcctgagcgataacgccaccgccttcagcaacagaagcaagcagctgcggagacagatgtggtggcggggctgcaagattaaggccatcatggctctggtggccgccatcctgctgctggtcatcatcatcctgatcgtgatgaagtaccggacaggcggcggaggatctggcggaggtggaagcggaggcggaggaagtggatctattggagccgccagcatggaattttgcttcgacgtgttcaaagaactgaaggtgcaccacgccaacgagaacatcttctactgccctatcgccatcatgagcgccctggctatggtgtatctgggcgccaaggacagcacccggacacagatcaacaaggtcgtcagattcgacaagctgcccggcttcggcgattctatcgaagcccagtgtggcaccagcgtgaacgtgcacagcagcctgagagacatcctgaatcagatcaccaagcctaacgacgtgtactccttcagcctggccagcagactgtacgccgaggaaagataccccatcctgcctgagtacctgcagtgcgtgaaagagctgtacagaggcggcctggaacctatcaacttccagacagccgccgaccaggccagagagctgatcaattcttgggtcgagagccagaccaacggcatcatcagaaacgtgctgcagcccagctccgtggattctcagacagccatggtgctggtcaacgccattgtgtttaaaggcctgtgggagaaaaccttcaaggacgaggacacccaggccatgcctttcagagtgacagagcaagagtccaagcctgtgcagatgatgtaccagatcggcctgtttagagtggcctccatggcctccgagaagatgaagatcctcgagctgcctttcgccagcggcaccatgtctatgctggtgctgctgcctgatgaggtgtccggactggaacagctcgagagcatcatcaacttcgagaagctgaccgagtggaccagcagcaacgtgatggaagaacggaagatcaaggtgtacctgcctcggatgaagatggaagagaagtacaacctgaccagcgtgctgatggctatgggcatcacagacgtgttctccagcagcgccaatctgagcggcatcagctctgccgagagcctgaagatttctcaggccgtgcatgctgcccacgccgagattaacgaagccggcagagaagttgtgggatctgccgaagcaggcgtggacgctgcttctgtgtctgaggaattccgggccgaccatccttttctgttctgcatcaagcacattgccaccaacgccgtgctgttctttggcagatgcgtgtccccttga

SEQ ID NO: 62 - DNA, 1503 bp, synthetic construct
  source 1..1503: mol_type = other DNA; note = VAMP8-OVA
atggaagaggctagtgaaggcggcggaaacgacagagtgcggaatctgcagtctgaggtggaaggcgtgaagaacatcatgacccagaacgtggaacggatcctggccagaggcgagaacctggaacacctgagaaacaagaccgaggacctggaagccaccagcgagcactttaagaccaccagccagaaggtggcccggaagttctggtggaagaatgtgaagatgatcgtgctgatctgcgtgatcgtgttcatcatcatcctgttcatcgtgctgttcgccaccggcgccttttctggcggcggaggatctggcggaggtggaagcggaggcggaggaagtggatctattggagccgccagcatggaattttgcttcgacgtgttcaaagaactgaaggtgcaccacgccaacgagaacatcttctactgccctatcgccatcatgagcgccctggctatggtgtatctgggcgccaaggacagcacccggacacagatcaacaaggtcgtcagattcgacaagctgcccggcttcggcgattctatcgaagcccagtgtggcaccagcgtgaacgtgcacagcagcctgagagacatcctgaatcagatcaccaagcctaacgacgtgtactccttcagcctggccagcagactgtacgccgaggaaagataccccatcctgcctgagtacctgcagtgcgtgaaagagctgtacagaggcggcctggaacctatcaacttccagacagccgccgaccaggccagagagctgatcaattcttgggtcgagagccagaccaacggcatcatcagaaacgtgctgcagcccagctccgtggattctcagacagccatggtgctggtcaacgccattgtgtttaaaggcctgtgggagaaaaccttcaaggacgaggacacccaggccatgcctttcagagtgacagagcaagagtccaagcctgtgcagatgatgtaccagatcggcctgtttagagtggcctccatggcctccgagaagatgaagatcctcgagctgcctttcgccagcggcaccatgtctatgctggtgctgctgcctgatgaggtgtccggactggaacagctcgagagcatcatcaacttcgagaagctgaccgagtggaccagcagcaacgtgatggaagaacggaagatcaaggtgtacctgcctcggatgaagatggaagagaagtacaacctgaccagcgtgctgatggctatgggcatcacagacgtgttctccagcagcgccaatctgagcggcatcagctctgccgagagcctgaagatttctcaggccgtgcatgctgcccacgccgagattaacgaagccggcagagaagttgtgggatctgccgaagcaggcgtggacgctgcttctgtgtctgaggaattccgggccgaccatccttttctgttctgcatcaagcacattgccaccaacgccgtgctgttctttggcagatgcgtgtccccttga

SEQ ID NO: 63 - DNA, 1899 bp, synthetic construct
  source 1..1899: mol_type = other DNA; note = VTI1B-OVA
atggctagctctgccgccagctctgagcacttcgagaagctgcacgagatcttcagaggcctgcacgaggacctgcagggcgttccagaaagactgctgggaacagccggcaccgaggaaaagaagaagctgatccgggacttcgacgagaagcagcaagaggccaatgagacactggccgagatggaagaggaactgagatacgcccctctgagcttcagaaaccccatgatgagcaagctgcggaactaccggaaggacctggccaagctgcatagagaagtgcggagcacccctctgacagctacacctggtggaagaggcgacatgaagtacggcatctacgccgtggaaaacgagcacatgaaccggctgcagagccagagagctatgctgctgcagggcaccgagagcctgaatagagccacacagagcatcgagcggagccacagaatcgccaccgagacagatcagatcggcagcgagatcatcgaggaactgggcgagcagagggaccagctggaaaggaccaagagcagactggtcaacaccagcgagaacctgagcaagagccggaagatcctgcggagcatgagcagaaaagtgaccaccaacaagctgctgctgagcatcatcatcctgctggaactggccatcctcggcggcctggtgtactacaagttcttcagaagccatggcggcggaggatctggcggaggtggaagcggaggcggaggaagtggatctattggagccgccagcatggaattttgcttcgacgtgttcaaagaactgaaggtgcaccacgccaacgagaacatcttctactgccctatcgccatcatgagcgccctggctatggtgtatctgggcgccaaggacagcacccggacacagatcaacaaggtcgtcagattcgacaagctgcccggcttcggcgattctatcgaagcccagtgtggcaccagcgtgaacgtgcacagcagcctgagagacatcctgaatcagatcaccaagcctaacgacgtgtactccttcagcctggccagcagactgtacgccgaggaaagataccccatcctgcctgagtacctgcagtgcgtgaaagagctgtacagaggcggcctggaacctatcaacttccagacagccgccgaccaggccagagagctgatcaattcttgggtcgagagccagaccaacggcatcatcagaaacgtgctgcagcccagctccgtggattctcagacagccatggtgctggtcaacgccattgtgtttaaaggcctgtgggagaaaaccttcaaggacgaggacacccaggccatgcctttcagagtgacagagcaagagtccaagcctgtgcagatgatgtaccagatcggcctgtttagagtggcctccatggcctccgagaagatgaagatcctcgagctgcctttcgccagcggcaccatgtctatgctggtgctgctgcctgatgaggtgtccggactggaacagctcgagagcatcatcaacttcgagaagctgaccgagtggaccagcagcaacgtgatggaagaacggaagatcaaggtgtacctgcctcggatgaagatggaagagaagtacaacctgaccagcgtgctgatggctatgggcatcacagacgtgttctccagcagcgccaatctgagcggcatcagctctgccgagagcctgaagatttctcaggccgtgcatgctgcccacgccgagattaacgaagccggcagagaagttgtgggatctgccgaagcaggcgtggacgctgcttctgtgtctgaggaattccgggccgaccatccttttctgttctgcatcaagcacattgccaccaacgccgtgctgttctttggcagatgcgtgtccccttga

SEQ ID NO: 64 - DNA, 1953 bp, synthetic construct
  source 1..1953: mol_type = other DNA; note = GOSR1-OVA
atggccgctggcacaagcagctactgggaagatctgcggaagcaggcccggcagctggaaaatgagctggacctgaagctggtgtccttcagcaagctgtgcaccagctacagccacagcagcaccagagatggcagacgggacagatacagcagcgacaccacacctctgctgaacggcagcagccaggaccggatgtttgagacaatggccatcgagatcgaacagctgctggccagactgaccggcgtgaacgataagatggccgagtacaccaactctgccggcgtgccaagtctgaacgccgctctgatgcacaccctgcagagacacagagacattctgcaggactacacccacgagttccacaagaccaaggccaacttcatggccattcgcgagcgcgagaatctgatgggctctgtgcggaaggacatcgagagctacaagagcggctctggcgtgaacaacagacggaccgagctgttcctgaaagagcacgaccacctgagaaacagcgaccggctgatcgaggaaaccatctctatcgccatggccaccaaagaaaacatgaccagccagcggggcatgctgaagtccatccacagcaagatgaacaccctggccaacagattccccgccgtgaacagcctgatccagcggatcaatctgagaaagcggcgggactctctgatcctcggcggagtgatcggcatctgtaccatcctgctgctgctctacgccttccatggcggcggaggatctggcggaggtggaagcggaggcggaggaagtggatctattggagccgccagcatggaattttgcttcgacgtgttcaaagaactgaaggtgcaccacgccaacgagaacatcttctactgccctatcgccatcatgagcgccctggctatggtgtatctgggcgccaaggacagcacccggacacagatcaacaaggtcgtcagattcgacaagctgcccggcttcggcgattctatcgaagcccagtgtggcaccagcgtgaacgtgcacagcagcctgagagacatcctgaatcagatcaccaagcctaacgacgtgtactccttcagcctggccagcagactgtacgccgaggaaagataccccatcctgcctgagtacctgcagtgcgtgaaagagctgtacagaggcggcctggaacctatcaacttccagacagccgccgaccaggccagagagctgatcaattcttgggtcgagagccagaccaacggcatcatcagaaacgtgctgcagcccagctccgtggattctcagacagccatggtgctggtcaacgccattgtgtttaaaggcctgtgggagaaaaccttcaaggacgaggacacccaggccatgcctttcagagtgacagagcaagagtccaagcctgtgcagatgatgtaccagatcggcctgtttagagtggcctccatggcctccgagaagatgaagatcctcgagctgcctttcgccagcggcaccatgtctatgctggtgctgctgcctgatgaggtgtccggactggaacagctcgagagcatcatcaacttcgagaagctgaccgagtggaccagcagcaacgtgatggaagaacggaagatcaaggtgtacctgcctcggatgaagatggaagagaagtacaacctgaccagcgtgctgatggctatgggcatcacagacgtgttctccagcagcgccaatctgagcggcatcagctctgccgagagcctgaagatttctcaggccgtgcatgctgcccacgccgagattaacgaagccggcagagaagttgtgggatctgccgaagcaggcgtggacgctgcttctgtgtctgaggaattccgggccgaccatccttttctgttctgcatcaagcacattgccaccaacgccgtgctgttctttggcagatgcgtgtccccttga

SEQ ID NO: 65 - DNA, 1557 bp, synthetic construct
  source 1..1557: mol_type = other DNA; note = BET1-OVA
atgcggagagccggacttggagaaggtgtccctcctggcaactacggcaattacggctacgccaacagcggctactctgcctgcgaggaagagaacgagagactgaccgagagcctgcggagcaaagtgaccgccatcaagagcctgagcatcgagatcggccacgaagtgaaaacccagaacaagctgctggccgagatggacagccagttcgacagcaccacaggctttctgggcaagaccatgggcaagctgaagatcctgagcagaggcagccagacaaagctgctgtgctacatgatgctgttcagcctgttcgtgttcttcatcatctactggatcatcaagctgagaggcggcggaggatctggcggaggtggaagcggaggcggaggaagtggatctattggagccgccagcatggaattttgcttcgacgtgttcaaagaactgaaggtgcaccacgccaacgagaacatcttctactgccctatcgccatcatgagcgccctggctatggtgtatctgggcgccaaggacagcacccggacacagatcaacaaggtcgtcagattcgacaagctgcccggcttcggcgattctatcgaagcccagtgtggcaccagcgtgaacgtgcacagcagcctgagagacatcctgaatcagatcaccaagcctaacgacgtgtactccttcagcctggccagcagactgtacgccgaggaaagataccccatcctgcctgagtacctgcagtgcgtgaaagagctgtacagaggcggcctggaacctatcaacttccagacagccgccgaccaggccagagagctgatcaattcttgggtcgagagccagaccaacggcatcatcagaaacgtgctgcagcccagctccgtggattctcagacagccatggtgctggtcaacgccattgtgtttaaaggcctgtgggagaaaaccttcaaggacgaggacacccaggccatgcctttcagagtgacagagcaagagtccaagcctgtgcagatgatgtaccagatcggcctgtttagagtggcctccatggcctccgagaagatgaagatcctcgagctgcctttcgccagcggcaccatgtctatgctggtgctgctgcctgatgaggtgtccggactggaacagctcgagagcatcatcaacttcgagaagctgaccgagtggaccagcagcaacgtgatggaagaacggaagatcaaggtgtacctgcctcggatgaagatggaagagaagtacaacctgaccagcgtgctgatggctatgggcatcacagacgtgttctccagcagcgccaatctgagcggcatcagctctgccgagagcctgaagatttctcaggccgtgcatgctgcccacgccgagattaacgaagccggcagagaagttgtgggatctgccgaagcaggcgtggacgctgcttctgtgtctgaggaattccgggccgaccatccttttctgttctgcatcaagcacattgccaccaacgccgtgctgttctttggcagatgcgtgtccccttga

SEQ ID NO: 66 - DNA, 2073 bp, synthetic construct
  source 1..2073: mol_type = other DNA; note = BET1L-OVA
atggccttttgcgccatcctgctggtgcctagcctgtgcagaatgcccagcctgcctacaagcccttgggcctttcctgtgcattgggccggcttcatgttcaagcccctggactggcagggcaacgacttcttcccacctcaagacgaagtgctggccccttgcctgggcatcaagacacctctgaagcacgagccctgtgctagcctgcctttcagcgtgctgtttcagagcagcgccagccagtctctgctgggcacaatgggatctctgagccctcacctgtgcggccacacaatgtgccctgtgaatcctgagctgccactgagcttccaggccgaccatagatctgcccagccagatgcctgcagtcccctgtgtcatccatctagcctgctgcctagcttccacaccgcttctctgcccttcagcattcacgcccaccactctccactgccttgcgaccttgatcctcctctgtacctggccgagacagtgtccctgctggaagaatggggacctcctagcagctgccccatgcagtgcaagctgacatctcaccctgccagactgacccatctgcctccatgtctgtggggctttgccgtggctctgaagccttcttgggctggccttgctccttctctgctgcctccacctagaatgagcctgtgtagacccctgtccttcctgcggcatcagtgtccttggctgccttggcaggctcaccaaggacttgttccttggagcccctctatggtggccgctgcctgtatcgtgtctcctagcggacactgtagatgccagcctttcatccctcacgtgttcctcggacacggcggcctgacatctgtgtctggcgaatgcggaggcggcggaggatctggcggaggtggaagcggaggcggaggaagtggatctattggagccgccagcatggaattttgcttcgacgtgttcaaagaactgaaggtgcaccacgccaacgagaacatcttctactgccctatcgccatcatgagcgccctggctatggtgtatctgggcgccaaggacagcacccggacacagatcaacaaggtcgtcagattcgacaagctgcccggcttcggcgattctatcgaagcccagtgtggcaccagcgtgaacgtgcacagcagcctgagagacatcctgaatcagatcaccaagcctaacgacgtgtactccttcagcctggccagcagactgtacgccgaggaaagataccccatcctgcctgagtacctgcagtgcgtgaaagagctgtacagaggcggcctggaacctatcaacttccagacagccgccgaccaggccagagagctgatcaattcttgggtcgagagccagaccaacggcatcatcagaaacgtgctgcagcccagctccgtggattctcagacagccatggtgctggtcaacgccattgtgtttaaaggcctgtgggagaaaaccttcaaggacgaggacacccaggccatgcctttcagagtgacagagcaagagtccaagcctgtgcagatgatgtaccagatcggcctgtttagagtggcctccatggcctccgagaagatgaagatcctcgagctgcctttcgccagcggcaccatgtctatgctggtgctgctgcctgatgaggtgtccggactggaacagctcgagagcatcatcaacttcgagaagctgaccgagtggaccagcagcaacgtgatggaagaacggaagatcaaggtgtacctgcctcggatgaagatggaagagaagtacaacctgaccagcgtgctgatggctatgggcatcacagacgtgttctccagcagcgccaatctgagcggcatcagctctgccgagagcctgaagatttctcaggccgtgcatgctgcccacgccgagattaacgaagccggcagagaagttgtgggatctgccgaagcaggcgtggacgctgcttctgtgtctgaggaattccgggccgaccatccttttctgttctgcatcaagcacattgccaccaacgccgtgctgttctttggcagatgcgtgtccccttga

SEQ ID NO: 67 - DNA, 1848 bp, synthetic construct
  source 1..1848: mol_type = other DNA; note = SEC22B-OVA
atggtcctgctgaccatgattgccagagtggccgatggactgcctctggccgctagcatgcaagaggatgagcagagcggcagagatctgcagcagtaccagtctcaggccaagcagctgttccggaagctgaacgagcagagccctaccagatgcacccttgaagccggcgctatgaccttccactacatcatcgagcagggcgtgtgctacctggtgctgtgcgaagccgcctttcctaagaagctggccttcgcctacctggaagatctgcacagcgagttcgatgagcagcacggcaagaaggtgcccaccgtcagcagaccctacagcttcatcgagttcgacaccttcatccaaaagaccaagaagctgtacatcgacagccgggccagaagaaacctgggcagcatcaataccgagctgcaggacgtgcagagaatcatggtggccaacatcgaggaagtgctgcagagaggcgaagccctgtctgccctggatagcaaggccaacaatctgagcagcctgagcaagaagtaccggcaggacgccaagtacctgaacatgagaagcacctacgccaagctggccgccgtggccgtgttcttcatcatgctgatcgtgtacgtgcggttctggtggcttggcggcggaggatctggcggaggtggaagcggaggcggaggaagtggatctattggagccgccagcatggaattttgcttcgacgtgttcaaagaactgaaggtgcaccacgccaacgagaacatcttctactgccctatcgccatcatgagcgccctggctatggtgtatctgggcgccaaggacagcacccggacacagatcaacaaggtcgtcagattcgacaagctgcccggcttcggcgattctatcgaagcccagtgtggcaccagcgtgaacgtgcacagcagcctgagagacatcctgaatcagatcaccaagcctaacgacgtgtactccttcagcctggccagcagactgtacgccgaggaaagataccccatcctgcctgagtacctgcagtgcgtgaaagagctgtacagaggcggcctggaacctatcaacttccagacagccgccgaccaggccagagagctgatcaattcttgggtcgagagccagaccaacggcatcatcagaaacgtgctgcagcccagctccgtggattctcagacagccatggtgctggtcaacgccattgtgtttaaaggcctgtgggagaaaaccttcaaggacgaggacacccaggccatgcctttcagagtgacagagcaagagtccaagcctgtgcagatgatgtaccagatcggcctgtttagagtggcctccatggcctccgagaagatgaagatcctcgagctgcctttcgccagcggcaccatgtctatgctggtgctgctgcctgatgaggtgtccggactggaacagctcgagagcatcatcaacttcgagaagctgaccgagtggaccagcagcaacgtgatggaagaacggaagatcaaggtgtacctgcctcggatgaagatggaagagaagtacaacctgaccagcgtgctgatggctatgggcatcacagacgtgttctccagcagcgccaatctgagcggcatcagctctgccgagagcctgaagatttctcaggccgtgcatgctgcccacgccgagattaacgaagccggcagagaagttgtgggatctgccgaagcaggcgtggacgctgcttctgtgtctgaggaattccgggccgaccatccttttctgttctgcatcaagcacattgccaccaacgccgtgctgttctttggcagatgcgtgtccccttga

SEQ ID NO: 68 - DNA, 1980 bp, synthetic construct
  source 1..1980: mol_type = other DNA; note = USE1-OVA
atggccgcctctagactggaactgaatctcgtgcggctgctgagcagatgcgaagctatggccgccgagaagagggaccctgatgaatggcggctcgagaaatatgtgggcgccctggaagatatgctgcaggccctgaaagtgcacgccagcaagcctgccagcgaagtgatcaacgagtacagctggaaggtggacttcctgaagggcatgctccaggccgagaagctgacaagcagctctgaaaaggccctggccaaccagtttctggcccctggtagagtgcctaccaccgccagagaaagagtgccagccaccaagacagtgcacctccagagcagagccagatacaccagcgagatgagaagcgagctgctgggcacagattctgccgagcctgaaatggacgtgcggaagagaacaggcgtggcaggctctcagcctgtgtccgaaaaacagctggccgctgagctggatctggtgctgcagagacaccagaacctgcaagagaagctggccgaggaaatgctgggcctcgccagatctctgaaaacaaacaccctggccgctcagagcgtgatcaagaaggacaatcagaccctgagccacagcctgaagatggccgaccagaatctggaaaagctgaaaaccgagagcgagcggctggaacagcacacccagaaaagcgtgaactggctgctgtgggccatgctgatcatcgtgtgcttcatcttcatcagcatgatcctgttcatccggatcatgcccaagctgaaaggcggcggaggatctggcggaggtggaagcggaggcggaggaagtggatctattggagccgccagcatggaattttgcttcgacgtgttcaaagaactgaaggtgcaccacgccaacgagaacatcttctactgccctatcgccatcatgagcgccctggctatggtgtatctgggcgccaaggacagcacccggacacagatcaacaaggtcgtcagattcgacaagctgcccggcttcggcgattctatcgaagcccagtgtggcaccagcgtgaacgtgcacagcagcctgagagacatcctgaatcagatcaccaagcctaacgacgtgtactccttcagcctggccagcagactgtacgccgaggaaagataccccatcctgcctgagtacctgcagtgcgtgaaagagctgtacagaggcggcctggaacctatcaacttccagacagccgccgaccaggccagagagctgatcaattcttgggtcgagagccagaccaacggcatcatcagaaacgtgctgcagcccagctccgtggattctcagacagccatggtgctggtcaacgccattgtgtttaaaggcctgtgggagaaaaccttcaaggacgaggacacccaggccatgcctttcagagtgacagagcaagagtccaagcctgtgcagatgatgtaccagatcggcctgtttagagtggcctccatggcctccgagaagatgaagatcctcgagctgcctttcgccagcggcaccatgtctatgctggtgctgctgcctgatgaggtgtccggactggaacagctcgagagcatcatcaacttcgagaagctgaccgagtggaccagcagcaacgtgatggaagaacggaagatcaaggtgtacctgcctcggatgaagatggaagagaagtacaacctgaccagcgtgctgatggctatgggcatcacagacgtgttctccagcagcgccaatctgagcggcatcagctctgccgagagcctgaagatttctcaggccgtgcatgctgcccacgccgagattaacgaagccggcagagaagttgtgggatctgccgaagcaggcgtggacgctgcttctgtgtctgaggaattccgggccgaccatccttttctgttctgcatcaagcacattgccaccaacgccgtgctgttctttggcagatgcgtgtccccttga

SEQ ID NO: 69 - DNA, 1881 bp, synthetic construct
  source 1..1881: mol_type = other DNA; note = VAMP7-pc-OVA
atggccatcctgttcgccgtggtggctagaggcacaaccattctggccaagcacgcttggtgcggcggcaactttctggaagtgaccgagcagatcctggccaagattcccagcgagaacaacaagctgacctacagccacggcaactacctgttccactacatctgccaggaccggatcgtgtacctgtgcatcaccgacgacgacttcgagcggagcagagccttcaacttcctgaacgagatcaagaagcggttccagaccacctacggcagcagagcacaaacagccctgccttacgccatgaacagcgagttcagctctgtgctggccgctcagctgaagcaccactccgagaacaaaggcctggacaaagtgatggaaacacaggcccaggtggacgagctgaagggcatcatggtccgaaacatcgacctggtggcccagagaggcgagagactggaactgctgatcgacaagaccgagaacctggtggacagcagcgtgaccttcaagaccaccagcagaaacctggccagagccatgtgcatgaagaacctgaagctgacgatcatcatcattatcgtgtccatcgtgttcatctacatcatcgtgtccccactgtgtggcggcttcacctggcctagctgtgtgaagaaatctggcggcggaggatctggcggaggtggaagcggaggcggtggatctagaagggccagaagaggatctatcggagccgccagcatggaattttgcttcgacgtgttcaaagaactgaaggtgcaccacgccaacgagaacatcttctactgccctatcgccatcatgagcgccctggctatggtgtatctgggcgccaaggacagcacccggacacagatcaacaaggtcgtcagattcgacaagctgcccggcttcggcgattctatcgaagcccagtgtggcaccagcgtgaacgtgcacagcagcctgagagacatcctgaatcagatcaccaagcctaacgacgtgtactccttcagcctggccagcagactgtacgccgaggaaagataccccatcctgcctgagtacctgcagtgcgtgaaagagctgtacagaggcggcctggaacctatcaacttccagacagccgccgaccaggccagagagctgatcaattcttgggtcgagagccagaccaacggcatcatcagaaacgtgctgcagcccagctccgtggattctcagacagccatggtgctggtcaacgccattgtgtttaaaggcctgtgggagaaaaccttcaaggacgaggacacccaggccatgcctttcagagtgacagagcaagagtccaagcctgtgcagatgatgtaccagatcggcctgtttagagtggcctccatggcctccgagaagatgaagatcctcgagctgcctttcgccagcggcaccatgtctatgctggtgctgctgcctgatgaggtgtccggactggaacagctcgagagcatcatcaacttcgagaagctgaccgagtggaccagcagcaacgtgatggaagaacggaagatcaaggtgtacctgcctcggatgaagatggaagagaagtacaacctgaccagcgtgctgatggctatgggcatcacagacgtgttctccagcagcgccaatctgagcggcatcagctctgccgagagcctgaagatttctcaggccgtgcatgctgcccacgccgagattaacgaagccggcagagaagttgtgggatctgccgaagcaggcgtggacgctgcttctgtgtctgaggaattccgggccgaccatccttttctgttctgcatcaagcacattgccaccaacgccgtgctgttctttggcagatgcgtgtccccttga

SEQ ID NO: 70 - DNA, 2409 bp, synthetic construct
  source 1..2409: mol_type = other DNA; note = LAMP[OVA]
atggctgcccctggctctgctagaaggcctctgctgttgctgcttctgctgctgctcctgggcctgatgcattgtgcctctgccgccatgttcatggtcaagaacggcaatggcaccgcctgcatcatggccaatttcagcgccgccttcagcgtgaactacgacaccaagagcggccccaagaacatgaccttcgacctgccttctgacgccaccgtggtgctgaatagaagcagctgcggcaaagagaacaccagcgatcccagcctcgtgatcgcctttggcagaggccatacactgaccctgaacttcacccggaacgccaccagatacagcgtgcagctgatgagcttcgtgtacaacctgagcgacacccatctgttccccaacgccagcagcaaagagatcaagaccgtcgagagcatcaccgacatccgggccgacatcgacaaaaagtacagatgcgtgtccggcacacaggtgcacatgaacaacgtgaccgtgacactgcacgacgccaccatccaggcctacctgagcaacagctctttcagcaggggcgagacaagatgcgagcaggacagaccctctcctaccactgctcctccagctccaccttctccaagtccatctcctgtgcctaagagccccagcgtggacaagtacaatgtgtctggcaccaacggcacctgtctgctggcttctatgggcctgcagctgaacctgacctacgagcggaaggacaacaccaccgtgaccagactgctgaacatcaaccccaacaagaccagcgccagcggatcttgtggcgcccatctggttacactggaactgcacagcgagggcaccacagtgctgctgttccagttcggcatgaacgccagctccagccggttcttcctgcaaggcatccagctgaacaccatcctgcctgacgccagagatcctgccttcaaggccgccaatggaagcctgagagcactgcaggccacagtgggcaacagctacaagtgcaacgccgaggaacacgtgcgcgtgaccaaggccttctccgtgaacatcttcaaagtgtgggtgcaagcctttaaggtggaaggcggccagtttggcagcgtggaagaatgcctgctggacgagaatagcatgggctctatcggagccgccagcatggaattttgcttcgacgtgttcaaagagctgaaggtccaccacgccaacgagaatatcttctactgccctatcgccatcatgagcgccctggccatggtgtatctgggcgccaaggatagcacccggacacagatcaacaaggtcgtcagattcgacaagctgcccggcttcggcgattctatcgaagcccagtgtggcacctccgtgaatgtgcacagcagcctgagggacatcctgaaccagatcaccaagcctaacgacgtgtacagcttcagcctggcctccagactgtacgccgaagagagataccccattctgcccgagtacctgcagtgtgtgaaagaactgtacagaggcggcctggaacctatcaacttccagacagccgccgaccaggccagagagctgatcaattcttgggtcgagagccagaccaatggcatcatccggaacgtgctgcagcccagctctgtggattctcagactgccatggtgctggtcaacgccatcgtgtttaaaggcctgtgggagaaaaccttcaaggacgaggacacccaggccatgcctttcagagtgaccgagcaagagtccaagcctgtgcagatgatgtaccagatcggcctgtttagagtggcctccatggcctccgagaagatgaagatcctcgagctgcctttcgccagcggcaccatgtctatgttggtgctgctgcccgatgaggtgtccggactggaacaactggaatccatcatcaacttcgagaagctgaccgagtggaccagctccaacgtgatggaagaacggaagatcaaggtgtacctgcctcggatgaagatggaagagaagtacaatctgaccagcgtgctgatggccatgggaatcaccgatgtgttctccagcagcgccaacctgtctggcatcagctctgccgagagcctgaagatttctcaggccgtgcatgccgctcacgccgagatcaatgaagccggcagagaagttgtgggatctgccgaagcaggcgtggacgctgcatctgtgtctgaggaattcagagccgaccatccttttctgttctgcatcaagcacattgccaccaacgccgtgctgttcttcggaagatgtgtgtcccctctgatcccaatcgccgttggaggtgctctggctggactggtgctgatcgtgctgattgcctacctcgtgggcagaaagagaagccacgccggctaccagaccatctga

SEQ ID NO: 71 - DNA, 753 bp, Homo sapiens
  source 1..753: mol_type = genomic DNA
atggcggcagggaccagcagttactgggaagatctcaggaaacaggctcgacagctggaaaatgaacttgacctgaaactagtttccttcagcaaactatgtacaagttacagtcatagcagtacccgagatggaagacgcgacaggtatagttctgatacaacaccccttttaaatggatcaagccaagacagaatgtttgagacaatggcgattgagattgaacaacttttggcaaggcttacaggggtaaatgataaaatggcagaatataccaacagtgcaggtgtcccctccttgaatgcagccctgatgcatacattacagcggcatagagacatattgcaggattatacacatgaattccataaaaccaaagcaaactttatggcaatacgggaaagggagaatcttatgggatcagtacgaaaagatattgagtcatataaaagtgggtctggagtaaacaacagaagaactgagctatttttgaaagaacatgaccaccttcgaaactcagatcgtctgatagaagagacaataagcattgctatggcaacaaaagaaaatatgacttcacagagaggaatgttgaagtcaattcacagcaaaatgaacactttggccaatcgttttcctgctgtaaacagcctgatccagaggatcaacctgaggaagcggcgggactcgctcatcctagggggtgttattgggatctgtaccatcctgttgctgctgtatgcgttccattga

SEQ ID NO: 72 - DNA, 711 bp, Homo sapiens
  source 1..711: mol_type = genomic DNA
atggcaccggacccctggttctccacatacgattctacttgtcaaattgcccaagaaattgctgagaaaattcaacaacgaaatcaatatgaaagaaaaggtgaaaaggcaccaaagcttaccgtgacaatcagagctttgttgcagaacctgaaggaaaagatcgcccttttgaaggacttattgctaagagctgtgtcaacacatcagataacacagcttgaaggggaccgaagacagaacctcttggatgatcttgtaactcgagagagactacttctggcatcctttaagaatgagggtgccgaaccagatctaatcaggtccagcctgatgagtgaagaggctaagcgaggagcacccaacccttggctctttgaggagccagaggagaccagaggcttgggttttgatgaaatccggcaacagcagcagaaaattatccaagaacaggacgcaggccttgatgccctttcctctatcataagtcgccaaaaacaaatggggcaggaaattgggaatgaattggatgaacaaaatgagataattgacgaccttgccaacctagtggagaacacagatgaaaaacttcgcaatgaaaccaggcgggtaaacatggtggacagaaagtcagcctcttgtgggatgatcatggtgattttactgctgcttgtggctatcgtggttgttgcagtctggccgaccaactga

SEQ ID NO: 73 - DNA, 831 bp, Homo sapiens
  source 1..831: mol_type = genomic DNA
atgtcatacggtcccttagacatgtaccggaacccggggccctcggggccccagctccgggacttcagcagcatcatccagacgtgcagcggcaacatccagcggatcagccaagccactgctcagataaagaatttgatgagccagctaggaactaagcaggactcaagcaagctacaggaaaatctgcaacagttacaacactccacaaatcagctcgccaaggaaacaaatgaattgctgaaagaattagggtccttgccccttcccttatctacttcagaacagcgccagcagagacttcagaaggaacgcctcatgaatgacttctctgcagccttaaacaatttccaggctgtgcagagaagggtatctgaaaaggaaaaggagagtattgccagagcaagagctggatctcgtctttctgcagaagagaggcaaagagaggagcagctggtctcatttgacagccatgaggagtggaaccagatgcagagccaggaggatgaggtggccatcactgagcaggatttggaacttattaaagaaagagaaacggcaattcggcagctggaggctgacattttggatgtcaatcagatatttaaagatttggccatgatgatccatgaccagggtgatctgattgatagcatagaagccaatgtggaaagctcagaggtgcacgtcgaaagagccactgaacagttacagcgagctgcttactatcagaaaaaatctcgcaagaagatgtgtatcctggtgcttgtcctgtcagtgattattctaatcttgggacttattatctggctagtttataaaacgaagtga

SEQ ID NO: 74 - DNA, 303 bp, Homo sapiens
  source 1..303: mol_type = genomic DNA
atggaggaagccagtgaaggtggaggaaatgatcgtgtgcggaacctgcaaagtgaggtggagggagttaagaatattatgacccagaatgtggagcggatcctggcccggggggaaaacttggaacatctccgcaacaagacagaggatctggaagccacatctgagcacttcaagacgacatcgcagaaggtggctcgaaaattctggtggaagaacgtgaagatgattgtccttatctgcgtgattgtttttatcatcatcctcttcattgtgctctttgccactggtgccttctcttaa

SEQ ID NO: 75 - DNA, 648 bp, Homo sapiens
  source 1..648: mol_type = genomic DNA
atggtgttgctaacaatgatcgcccgagtggcggacgggctcccgctggccgcctcgatgcaggaggacgaacagtctggccgggaccttcaacaatatcagagtcaggctaagcaactctttcgaaagttgaatgaacagtcccctaccagatgtaccttggaagcaggagccatgacttttcactacattattgagcagggggtgtgttatttggttttatgtgaagctgccttccctaagaagttggcttttgcctacctagaagatttgcactcagaatttgatgaacagcatggaaagaaggtgcccactgtgtcccgaccctattcctttattgaatttgatactttcattcagaaaaccaagaagctctacattgacagtcgtgctcgaagaaatctaggctccatcaacactgaattgcaagatgtgcagaggatcatggtggccaatattgaagaagtgttacaacgaggagaagcactctcagcattggattcaaaggctaacaatttgtccagtctgtccaagaaataccgccaggatgcgaagtacttgaacatgcgttccacttatgccaaacttgcagcagtagctgtatttttcatcatgttaatagtgtatgtccgattctggtggctgtga

SEQ ID NO: 76 - DNA, 768 bp, Homo sapiens
  source 1..768: mol_type = genomic DNA
atgtccatggaggaccccttctttgtggtgaaaggagaggtacagaaagcagtcaacactgcccagggattgtttcagagatggacagagctcctccaggacccctccacagcaacaagggaagaaatcgactggaccaccaacgagctgagaaataacctccggagcatagagtgggatctagaggaccttgatgaaaccatcagcatagttgaagcaaatcctagaaaatttaaccttgatgcaactgaattgagtataagaaaagccttcattacaagtactcggcaagttgtcagggacatgaaagatcagatgtcaacttcatctgtgcaggcattagctgaaagaaaaaatagacaggcactgctgggagacagtggcagccagaactggagcactggaacaacagataaatatgggcgtctggaccgagagctccagagagccaattctcatttcattgaggagcagcaggcacagcagcagttgatcgtggaacagcaggatgagcagttggagctggtctctggcagcatcggggtgctgaagaacatgtcccagcgcatcggaggggagctggaggaacaggcagttatgttggaagatttctctcacgaattggagagcactcagtcccggctggacaatgtgatgaagaaacttgcaaaagtatctcatatgaccagtgatcggcgccaatggtgtgccatagccatcctctttgcagtcctgttggttgtgctcatcctcttcttagtgctgtga

SEQ ID NO: 77 - DNA, 303 bp, Homo sapiens
  source 1..303: mol_type = genomic DNA
atgtctacaggtccaactgctgccactggcagtaatcgaagacttcagcagacacaaaatcaagtagatgaggtggtggacataatgcgagttaacgtggacaaggttctggaaagagaccagaagctctctgagttagacgaccgtgcagacgcactgcaggcaggcgcttctcaatttgaaacgagcgcagccaagttgaagaggaaatattggtggaagaattgcaagatgtgggcaatcgggattactgttctggttatcttcatcatcatcatcatcgtgtgggttgtctcttcatga

SEQ ID NO: 78 - DNA, 426 bp, Homo sapiens
  source 1..426: mol_type = genomic DNA
atgcctcccaagtttaagcgccacctcaatgatgatgatgtcacaggttctgtgaaaagtgaaaggagaaatcttttggaagatgattcagatgaagaagaggacttttttctaaggggaccatctggaccaagatttggacctagaaatgataaaattaagcatgttcagaatcaagtggatgaagttattgatgtcatgcaagaaaatattacaaaggtaattgagagaggggagagactagatgaactacaggacaaatcagaaagcttatcggataatgcaacagcttttagcaacagatccaaacaacttcgaaggcaaatgtggtggcgtggatgcaaaataaaagccatcatggctttggttgctgctatccttttgctagtgattatcattcttatagtcatgaaataccgtacttga

SEQ ID NO: 79 - DNA, 699 bp, Homo sapiens
  source 1..699: mol_type = genomic DNA
atggcctcctccgccgcctcctcggagcatttcgagaagctgcacgagatcttccgcggcctccatgaagacctacaaggggtgcccgagcggctgctggggacggcggggaccgaagaaaagaagaaattgatcagggattttgatgaaaagcaacaggaagcaaatgaaacgctggcagagatggaggaggagctacgttatgcacccctgtctttccgaaaccccatgatgtctaagcttcgaaactaccggaaggaccttgctaaactccatcgggaggtgagaagcacacctttgacagccacacctggaggccgaggagacatgaaatatggcatatatgctgtagagaatgagcatatgaatcggctacagtctcaaagggcaatgcttctgcagggcactgaaagcctgaaccgggccacccaaagtattgaacgttctcatcggattgccacagagactgaccagattggctcagaaatcatagaagagctgggggaacaacgagaccagttagaacgtaccaagagtagactggtaaacacaagtgaaaacttgagcaaaagtcggaagattctccgttcaatgtccagaaaagtgacaaccaacaagctgctgctttccattatcatcttactggagctcgccatcctgggaggcctggtttactacaaattctttcgcagccattga

SEQ ID NO: 80 - DNA, 357 bp, Homo sapiens
  source 1..357: mol_type = genomic DNA
atgaggcgtgcaggcctgggtgaaggagtacctcctggcaactatgggaactatggctatgctaatagtgggtatagtgcctgtgaagaagaaaatgagaggctcactgaaagtctgagaagcaaagtaactgctataaaatctctttccattgaaataggccatgaagttaaaacccagaataaattattagctgaaatggattcacaatttgattccacaactggatttctaggtaaaactatgggcaaactgaagattttatccagagggagccaaacaaagctgctgtgctatatgatgctgttttctttatttgtcttttttatcatttattggattattaaactgaggtga

SEQ ID NO: 81 - DNA, 873 bp, Homo sapiens
  source 1..873: mol_type = genomic DNA
atggcattctgtgccatcctccttgtccccagcctctgcaggatgccctccttacccacctctccctgggccttccctgtccactgggctggattcatgttcaaaccactggactggcagggcaacgacttcttcccacctcaagatgaggtcctcgccccttgtcttggcataaaaacacctttaaagcatgagccatgtgcttctttgcccttttctgtcctgttccaatcttctgcctcccagtcactcctggggactatgggatcactgtccccccacctgtgtggccacaccatgtgtcctgtcaatccagaactgcctctgagcttccaggctgaccacagatcagcacagcctgatgcctgcagcccactttgtcacccttcctcccttcttccttccttccacacagcaagcctacctttctccatccatgctcaccatagcccccttccttgtgacctggaccctccattgtacctggctgagactgtcagcctcctggaggagtggggtccaccttcttcttgccctatgcagtgcaagctcacttctcacccagcaaggttgactcatctgcctccatgtctctggggctttgctgttgccctgaaacctagctgggctggtcttgctcccagcttgcttccccctcctcggatgtccctttgcaggcccctgtcgttcctccggcaccagtgtccttggctgccatggcaagctcatcaggggcttgtaccctggtcaccaagcatggtagcagctgcctgcattgtatctccatctggtcactgcaggtgccaacccttcatcccccatgttttcctgggccatggagggctgacctccgtttctggggaatgtggctga

SEQ ID NO: 82 - DNA, 780 bp, Homo sapiens
  source 1..780: mol_type = genomic DNA
atggcggcgtcgaggctggagctaaacctggtgcggctgctatcccgctgcgaggcgatggcagcggagaaacgggacccggacgagtggcgcctggagaagtacgtgggagccctagaggacatgttgcaggccctgaaggtccacgcgagcaaaccggcctctgaggtgatcaatgaatattcctggaaggtggattttctgaaggggatgctgcaagccgagaagctgacctcctcctcagagaaagcactggccaaccagttcctggcccctggccgtgtgccaaccacagccagagagcgagtgcccgccacaaagacggtgcatctgcagtcacgggcgcggtacaccagcgagatgcggagtgagctactaggcacggactctgcagagcctgagatggacgtaaggaagagaactggagtggcagggtcccagccagtgagtgagaagcagttggcagctgagctagacctcgtcctgcagcgacatcagaacctccaggaaaagctggcggaagagatgctaggactggcccggagcctcaagaccaataccctggccgcccagagtgtcatcaagaaggacaaccagaccctgtcacactcactgaaaatggcggaccagaacctggagaaactgaagacggagtcagagcgtctggagcagcacacgcagaagtcagtcaactggctgctctgggccatgctcattatcgtctgcttcatcttcattagcatgatcctcttcattcgaatcatgcctaaactcaaataa

SEQ ID NO: 83 - protein, 250 aa, Homo sapiens
MAAGTSSYWEDLRKQARQLENELDLKLVSFSKLCTSYSHSSTRDGRRDRYSSDTTPLLNGSSQDRMFETMAIEIEQLLARLTGVNDKMAEYTNSAGVPSLNAALMHTLQRHRDILQDYTHEFHKTKANFMAIRERENLMGSVRKDIESYKSGSGVNNRRTELFLKEHDHLRNSDRLIEETISIAMATKENMTSQRGMLKSIHSKMNTLANRFPAVNSLIQRINLRKRRDSLILGGVIGICTILLLLYAFH

SEQ ID NO: 84 - protein, 236 aa, Homo sapiens
MAPDPWFSTYDSTCQIAQEIAEKIQQRNQYERKGEKAPKLTVTIRALLQNLKEKIALLKDLLLRAVSTHQITQLEGDRRQNLLDDLVTRERLLLASFKNEGAEPDLIRSSLMSEEAKRGAPNPWLFEEPEETRGLGFDEIRQQQQKIIQEQDAGLDALSSIISRQKQMGQEIGNELDEQNEIIDDLANLVENTDEKLRNETRRVNMVDRKSASCGMIMVILLLLVAIVVVAVWPTN

SEQ ID NO: 85 - protein, 276 aa, Homo sapiens
MSYGPLDMYRNPGPSGPQLRDFSSIIQTCSGNIQRISQATAQIKNLMSQLGTKQDSSKLQENLQQLQHSTNQLAKETNELLKELGSLPLPLSTSEQRQQRLQKERLMNDFSAALNNFQAVQRRVSEKEKESIARARAGSRLSAEERQREEQLVSFDSHEEWNQMQSQEDEVAITEQDLELIKERETAIRQLEADILDVNQIFKDLAMMIHDQGDLIDSIEANVESSEVHVERATEQLQRAAYYQKKSRKKMCILVLVLSVIILILGLIIWLVYKTK

SEQ ID NO: 86 - protein, 100 aa, Homo sapiens
MEEASEGGGNDRVRNLQSEVEGVKNIMTQNVERILARGENLEHLRNKTEDLEATSEHFKTTSQKVARKFWWKNVKMIVLICVIVFIIILFIVLFATGAFS

SEQ ID NO: 87 - protein, 215 aa, Homo sapiens
MVLLTMIARVADGLPLAASMQEDEQSGRDLQQYQSQAKQLFRKLNEQSPTRCTLEAGAMTFHYIIEQGVCYLVLCEAAFPKKLAFAYLEDLHSEFDEQHGKKVPTVSRPYSFIEFDTFIQKTKKLYIDSRARRNLGSINTELQDVQRIMVANIEEVLQRGEALSALDSKANNLSSLSKKYRQDAKYLNMRSTYAKLAAVAVFFIMLIVYVRFWWL

SEQ ID NO: 88 - protein, 255 aa, Homo sapiens
MSMEDPFFVVKGEVQKAVNTAQGLFQRWTELLQDPSTATREEIDWTTNELRNNLRSIEWDLEDLDETISIVEANPRKFNLDATELSIRKAFITSTRQVVRDMKDQMSTSSVQALAERKNRQALLGDSGSQNWSTGTTDKYGRLDRELQRANSHFIEEQQAQQQLIVEQQDEQLELVSGSIGVLKNMSQRIGGELEEQAVMLEDFSHELESTQSRLDNVMKKLAKVSHMTSDRRQWCAIAILFAVLLVVLILFLVL

SEQ ID NO: 89 - protein, 100 aa, Homo sapiens
MSTGPTAATGSNRRLQQTQNQVDEVVDIMRVNVDKVLERDQKLSELDDRADALQAGASQFETSAAKLKRKYWWKNCKMWAIGITVLVIFIIIIIVWVVSS

SEQ ID NO: 90 - protein, 141 aa, Homo sapiens
MPPKFKRHLNDDDVTGSVKSERRNLLEDDSDEEEDFFLRGPSGPRFGPRNDKIKHVQNQVDEVIDVMQENITKVIERGERLDELQDKSESLSDNATAFSNRSKQLRRQMWWRGCKIKAIMALVAAILLLVIIILIVMKYRT

SEQ ID NO: 91 - protein, 232 aa, Homo sapiens
MASSAASSEHFEKLHEIFRGLHEDLQGVPERLLGTAGTEEKKKLIRDFDEKQQEANETLAEMEEELRYAPLSFRNPMMSKLRNYRKDLAKLHREVRSTPLTATPGGRGDMKYGIYAVENEHMNRLQSQRAMLLQGTESLNRATQSIERSHRIATETDQIGSEIIEELGEQRDQLERTKSRLVNTSENLSKSRKILRSMSRKVTTNKLLLSIIILLELAILGGLVYYKFFRSH

SEQ ID NO: 92 - protein, 118 aa, Homo sapiens
MRRAGLGEGVPPGNYGNYGYANSGYSACEEENERLTESLRSKVTAIKSLSIEIGHEVKTQNKLLAEMDSQFDSTTGFLGKTMGKLKILSRGSQTKLLCYMMLFSLFVFFIIYWIIKLR

SEQ ID NO: 93 - protein, 290 aa, Homo sapiens
MAFCAILLVPSLCRMPSLPTSPWAFPVHWAGFMFKPLDWQGNDFFPPQDEVLAPCLGIKTPLKHEPCASLPFSVLFQSSASQSLLGTMGSLSPHLCGHTMCPVNPELPLSFQADHRSAQPDACSPLCHPSSLLPSFHTASLPFSIHAHHSPLPCDLDPPLYLAETVSLLEEWGPPSSCPMQCKLTSHPARLTHLPPCLWGFAVALKPSWAGLAPSLLPPPRMSLCRPLSFLRHQCPWLPWQAHQGLVPWSPSMVAAACIVSPSGHCRCQPFIPHVFLGHGGLTSVSGECG

SEQ ID NO: 94 - protein, 259 aa, Homo sapiens
MAASRLELNLVRLLSRCEAMAAEKRDPDEWRLEKYVGALEDMLQALKVHASKPASEVINEYSWKVDFLKGMLQAEKLTSSSEKALANQFLAPGRVPTTARERVPATKTVHLQSRARYTSEMRSELLGTDSAEPEMDVRKRTGVAGSQPVSEKQLAAELDLVLQRHQNLQEKLAEEMLGLARSLKTNTLAAQSVIKKDNQTLSHSLKMADQNLEKLKTESERLEQHTQKSVNWLLWAMLIIVCFIFISMILFIRIMPKLK

SEQ ID NO: 95 - DNA, 1161 bp, synthetic construct
  source 1..1161: mol_type = other DNA
atgggctctatcggagccgccagcatggaattttgcttcgacgtgttcaaagagctgaaggtccaccacgccaacgagaacatcttctactgccctatcgccatcatgagcgccctggccatggtgtatctgggcgccaaggatagcacccggacacagatcaacaaggtcgtcagattcgacaagctgcccggcttcggcgattctatcgaagcccagtgtggcaccagcgtgaacgtgcacagcagcctgagagacatcctgaaccagatcaccaagcctaacgacgtgtacagcttcagcctggccagcagactgtacgccgaggaaagataccccatcctgcctgagtacctgcagtgcgtgaaagagctgtacagaggcggcctggaacctatcaacttccagacagccgccgaccaggccagagagctgatcaattcttgggtcgagagccagaccaacggcatcatcagaaacgtgctgcagcccagctccgtggattctcagacagccatggtgctggtcaacgccatcgtgtttaaaggcctgtgggagaaaaccttcaaggacgaggacacccaggccatgcctttcagagtgaccgagcaagagtccaagcctgtgcagatgatgtaccagatcggcctgtttagagtggcctccatggcctccgagaagatgaagatcctggaactgcctttcgccagcggcaccatgtctatgctggtgctgctgcctgatgaggtgtccggactggaacagctggaatccatcatcaacttcgagaagctgaccgagtggaccagcagcaacgtgatggaagaacggaagatcaaggtgtacctgcctcggatgaagatggaagagaagtacaacctgaccagcgtgctgatggccatgggaatcaccgatgtgttcagcagcagcgccaacctgagcggcattagctctgccgagagcctgaagattagccaggccgtgcatgctgcccacgccgagatcaatgaagccggcagagaagttgtgggatctgccgaagcaggcgtggacgctgcttctgtgtctgaggaattccgggccgaccatccttttctgttctgcatcaagcacattgccaccaacgccgtgctgttctttggcagatgcgtgtccccttga

SEQ ID NO: 96 - DNA, 1290 bp, Homo sapiens
  source 1..1290: mol_type = genomic DNA
atgggctccgacgtgcgggacctgaacgcgctgctgcccgccgtcccctccctgggtggcggcggcggctgtgccctgcctgtgagcggcgcggcgcagtgggcgccggtgctggactttgcgcccccgggcgcttcggcttacgggtcgttgggcggccccgcgccgccaccggctccgccgccacccccgccgccgccgcctcactccttcatcaaacaggagccgagctggggcggcgcggagccgcacgaggagcagtgcctgagcgccttcactgtccacttttccggccagttcactggcacagccggagcctgtcgctacgggcccttcggtcctcctccgcccagccaggcgtcatccggccaggccaggatgtttcctaacgcgccctacctgcccagctgcctcgagagccagcccgctattcgcaatcagggttacagcacggtcaccttcgacgggacgcccagctacggtcacacgccctcgcaccatgcggcgcagttccccaaccactcattcaagcatgaggatcccatgggccagcagggctcgctgggtgagcagcagtactcggtgccgcccccggtctatggctgccacacccccaccgacagctgcaccggcagccaggctttgctgctgaggacgccctacagcagtgacaatttataccaaatgacatcccagcttgaatgcatgacctggaatcagatgaacttaggagccaccttaaagggccacagcacagggtacgagagcgataaccacacaacgcccatcctctgcggagcccaatacagaatacacacgcacggtgtcttcagaggcattcaggatgtgcgacgtgtgcctggagtagccccgactcttgtacggtcggcatctgagaccagtgagaaacgccccttcatgtgtgcttacccaggctgcaataagagatattttaagctgtcccacttacagatgcacagcaggaagcacactggtgagaaaccataccagtgtgacttcaaggactgtgaacgaaggttttctcgttcagaccagctcaaaagacaccaaaggagacatacaggtgtgaaaccattccagtgtaaaacttgtcagcgaaagttctcccggtccgaccacctgaagacccacaccaggactcatacaggtgaaaagcccttcagctgtcggtggccaagttgtcagaaaaagtttgcccggtcagatgaattagtccgccatcacaacatgcatcagagaaacatgaccaaactccagctggcgctttga

SEQ ID NO: 97 - DNA, 1290 bp, synthetic construct
  source 1..1290: mol_type = other DNA
atgggcagcgacgtgcgggatctgaatgctctgcttcctgccgtgccatctcttggcggaggcggaggatgtgctttgcctgtttctggtgctgcccagtgggctcccgtgctggattttgctcctcctggcgcctctgcctatggctctcttggaggacctgctcctccaccagctccacctccaccgccgcctccaccacctcacagctttatcaagcaagagccctcctggggcggagccgaacctcatgaagaacagtgcctgagcgccttcaccgtgcacttcagcggacagtttacaggcacagccggcgcttgtagatacggcccttttggaccacctcctccaagccaggcttctagcggacaagcccggatgttccccaacgctccttacctgcctagctgcctggaaagccagcctgccatcagaaaccagggctacagcaccgtgaccttcgatggcacacctagctacggccacacaccatctcatcacgccgctcagttccccaatcacagcttcaagcacgaggaccctatgggccagcagggatctctgggagagcagcagtatagcgtgccacctcctgtgtacggctgtcacacccctaccgatagctgtacaggatctcaggccctgctgctgagaaccccttacagcagcgacaacctgtaccagatgaccagccagctggaatgcatgacctggaaccagatgaacctgggcgccacactgaagggccacagcacaggctacgagtccgacaaccacaccacacctattctgtgcggagcccagtaccggatccacacacatggcgtgttcagaggcatccaggacgtgcgaagagtgcctggcgttgcccctacactcgtcagatctgccagcgagacaagcgagaagcgccccttcatgtgtgcctatcctggctgcaacaagcggtacttcaagctgagccacctccagatgcacagcagaaagcacaccggcgagaagccctaccagtgcgacttcaaggactgcgagcggcggttcagcagaagcgaccagctgaaaagacaccagcggaggcacacaggcgtgaaacctttccagtgcaagacctgccagcggaagttctccagatccgatcacctgaaaacccacacacggacccacacaggggagaagccattcagctgtagatggcccagctgccagaagaagttcgctcggagcgacgaactcgtgcggcaccacaatatgcaccagagaaacatgaccaaactgcagctggccctgtga

SEQ ID NO: 98 - protein, 429 aa, Homo sapiens
MGSDVRDLNALLPAVPSLGGGGGCALPVSGAAQWAPVLDFAPPGASAYGSLGGPAPPPAPPPPPPPPPHSFIKQEPSWGGAEPHEEQCLSAFTVHFSGQFTGTAGACRYGPFGPPPPSQASSGQARMFPNAPYLPSCLESQPAIRNQGYSTVTFDGTPSYGHTPSHHAAQFPNHSFKHEDPMGQQGSLGEQQYSVPPPVYGCHTPTDSCTGSQALLLRTPYSSDNLYQMTSQLECMTWNQMNLGATLKGHSTGYESDNHTTPILCGAQYRIHTHGVFRGIQDVRRVPGVAPTLVRSASETSEKRPFMCAYPGCNKRYFKLSHLQMHSRKHTGEKPYQCDFKDCERRFSRSDQLKRHQRRHTGVKPFQCKTCQRKFSRSDHLKTHTRTHTGEKPFSCRWPSCQKKFARSDELVRHHNMHQRNMTKLQLAL

SEQ ID NO: 99 - DNA, 444 bp, synthetic construct
  source 1..444: mol_type = other DNA
atggaggtgggttggtaccgttctcccttctcaagagtggttcacctctaccgaaatggcaagatggaggtgggttggtaccgttctcccttctcaagagtggttcacctctaccgaaatggcaagatggaggtgggttggtaccgttctcccttctcaagagtggttcacctctaccgaaatggcaagatggaggtgggttggtaccgttctcccttctcaagagtggttcacctctaccgaaatggcaagatggaggtgggttggtaccgttctcccttctcaagagtggttcacctctaccgaaatggcaagatggaggtgggttggtaccgttctcccttctcaagagtggttcacctctaccgaaatggcaagatggaggtgggttggtaccgttctcccttctcaagagtggttcacctctaccgaaatggcaagtga

SEQ ID NO: 100 - DNA, 444 bp, synthetic construct
  source 1..444: mol_type = other DNA
atggaagtcggctggtatagaagccccttcagcagagtggtgcacctgtaccggaacggcaagatggaagttggatggtacaggtccccattcagccgggtcgtgcatctgtatagaaatggaaagatggaagttggctggtatcggagcccattttccagggtcgtccacctctacagaaacggcaaaatggaagtcggctggtacagatctccattctctagagtggtccatctctatcgcaacggaaagatggaagtcggatggtatcgctcccctttctctcgcgtggtgcatctttatcggaatggcaaaatggaagttggctggtataggtccccgttctccagagtcgttcacttgtataggaacggaaaaatggaagttggatggtatagatcacccttctctagggttgtgcacctctataggaatgggaagtga

SEQ ID NO: 101 - protein, 147 aa, synthetic construct
MEVGWYRSPFSRVVHLYRNGKMEVGWYRSPFSRVVHLYRNGKMEVGWYRSPFSRVVHLYRNGKMEVGWYRSPFSRVVHLYRNGKMEVGWYRSPFSRVVHLYRNGKMEVGWYRSPFSRVVHLYRNGKMEVGWYRSPFSRVVHLYRNGK

SEQ ID NO: 102 - DNA, 2010 bp, synthetic construct
  source 1..2010: mol_type = other DNA; note = VAMP7-pc-WT1
atggccatcctgttcgccgtggtggctagaggcacaaccattctggccaagcacgcttggtgcggcggcaactttctggaagtgaccgagcagatcctggccaagattcccagcgagaacaacaagctgacctacagccacggcaactacctgttccactacatctgccaggaccggatcgtgtacctgtgcatcaccgacgacgacttcgagcggagcagagccttcaacttcctgaacgagatcaagaagcggttccagaccacctacggcagcagagcacaaacagccctgccttacgccatgaacagcgagttcagctctgtgctggccgctcagctgaagcaccactccgagaacaaaggcctggacaaagtgatggaaacacaggcccaggtggacgagctgaagggcatcatggtccgaaacatcgacctggtggcccagagaggcgagagactggaactgctgatcgacaagaccgagaacctggtggacagcagcgtgaccttcaagaccaccagcagaaacctggccagagccatgtgcatgaagaacctgaagctgacgatcatcatcattatcgtgtccatcgtgttcatctacatcatcgtgtccccactgtgtggcggcttcacctggcctagctgtgtgaagaaatctggcggcggaggatctggcggaggtggaagcggaggcggtggatctagaagggctagaagaggctccgacgtgcgggacctgaatgctctgcttcctgccgtgccatctcttggcggtggtggtggatgtgcactgcctgtttctggtgctgctcagtgggctcccgtgctggattttgctcctcctggcgcctctgcctatggctctcttggaggacctgctcctccaccagctccaccgccacctccgcctccaccacctcacagctttatcaagcaagagccctcctggggcggagccgaacctcacgaagaacagtgtctgagcgccttcaccgtgcacttcagcggccagtttactggaacagccggcgcttgtagatacggcccttttggacctccacctcctagccaggcatctagcggacaggccaggatgttccccaacgctccttacctgccaagctgcctggaaagccagcctgccatcagaaaccagggctacagcaccgtgacattcgacggcacacctagctacggccacacaccttctcatcacgccgctcagttccccaatcacagcttcaagcacgaggaccccatgggccagcaaggatctttgggcgagcagcagtacagcgtgccacctcctgtgtacggctgtcacacccctaccgatagctgtacaggatctcaggccctgctgctgagaaccccttacagcagcgacaacctgtaccagatgaccagccagctggaatgcatgacctggaaccagatgaacctgggcgccacactgaagggccacagcacaggctacgagtccgacaaccacaccacacctattctgtgcggagcccagtaccggatccacacacatggcgtgttcagaggcatccaggacgtgcgaagagtgcctggcgttgcccctacactcgtcagatctgccagcgagacaagcgagaagcgccccttcatgtgtgcctatcctggctgcaacaagcggtacttcaagctgagccacctccagatgcacagcagaaagcacaccggcgagaagccctaccagtgcgacttcaaggactgcgagaggcggttcagcagaagcgaccagctgaagagacaccagcggagacatacaggcgtgaagcctttccagtgcaagacctgccagcggaagttctccagatccgaccacctgaaaacccacacaagaacccacaccggggaaaagccattcagctgcagatggcccagctgccagaagaagttcgctcggagcgacgaactcgtgcggcaccacaatatgcaccagagaaacatgaccaaactgcagctggccctgtga

SEQ ID NO: 103 - protein, 669 aa, synthetic construct
  source 1..669: note = VAMP7-pc-WT1
MAILFAVVARGTTILAKHAWCGGNFLEVTEQILAKIPSENNKLTYSHGNYLFHYICQDRIVYLCITDDDFERSRAFNFLNEIKKRFQTTYGSRAQTALPYAMNSEFSSVLAAQLKHHSENKGLDKVMETQAQVDELKGIMVRNIDLVAQRGERLELLIDKTENLVDSSVTFKTTSRNLARAMCMKNLKLTIIIIIVSIVFIYIIVSPLCGGFTWPSCVKKSGGGGSGGGGSGGGGSRRARRGSDVRDLNALLPAVPSLGGGGGCALPVSGAAQWAPVLDFAPPGASAYGSLGGPAPPPAPPPPPPPPPHSFIKQEPSWGGAEPHEEQCLSAFTVHFSGQFTGTAGACRYGPFGPPPPSQASSGQARMFPNAPYLPSCLESQPAIRNQGYSTVTFDGTPSYGHTPSHHAAQFPNHSFKHEDPMGQQGSLGEQQYSVPPPVYGCHTPTDSCTGSQALLLRTPYSSDNLYQMTSQLECMTWNQMNLGATLKGHSTGYESDNHTTPILCGAQYRIHTHGVFRGIQDVRRVPGVAPTLVRSASETSEKRPFMCAYPGCNKRYFKLSHLQMHSRKHTGEKPYQCDFKDCERRFSRSDQLKRHQRRHTGVKPFQCKTCQRKFSRSDHLKTHTRTHTGEKPFSCRWPSCQKKFARSDELVRHHNMHQRNMTKLQLAL

SEQ ID NO: 104 - DNA, 1167 bp, synthetic construct
  source 1..1167: mol_type = other DNA; note = VAMP7-pc-MOG 35-55
atggccatcctgttcgccgtggtggctagaggcacaaccattctggccaagcacgcttggtgcggcggcaactttctggaagtgaccgagcagatcctggccaagattcccagcgagaacaacaagctgacctacagccacggcaactacctgttccactacatctgccaggaccggatcgtgtacctgtgcatcaccgacgacgacttcgagcggagcagagccttcaacttcctgaacgagatcaagaagcggttccagaccacctacggcagcagagcacaaacagccctgccttacgccatgaacagcgagttcagctctgtgctggccgctcagctgaagcaccactccgagaacaaaggcctggacaaagtgatggaaacacaggcccaggtggacgagctgaagggcatcatggtccgaaacatcgacctggtggcccagagaggcgagagactggaactgctgatcgacaagaccgagaacctggtggacagcagcgtgaccttcaagaccaccagcagaaacctggccagagccatgtgcatgaagaacctgaagctgacgatcatcatcattatcgtgtccatcgtgttcatctacatcatcgtgtccccactgtgtggcggcttcacctggcctagctgtgtgaagaaatctggcggcggaggatctggcggaggtggaagcggaggcggtggatctagacgggctagaagaatggaagtcggctggtatcggagccccttcagcagagtggtgcacctgtaccggaacggcaagatggaagttggatggtacaggtccccattcagccgggtcgtgcatctgtatagaaatggaaagatggaagttggctggtatcgctctccattctccagagtggtccatctctaccgcaatggaaaaatggaagtcggatggtatagaagcccattctccagggttgtgcacctctacagaaacggaaaaatggaagtcggctggtacagatctcccttctctcgcgtggtgcatctttatcgcaacggaaagatggaagtcggatggtatcggtcaccttttagccgcgttgtccacctgtatcgtaatggcaaaatggaagttggatggtatcgctcacccttcagccgagtggttcatctctacagaaatggcaagtga

SEQ ID NO: 105 - protein, 388 aa, synthetic construct
  source 1..388: note = VAMP7-pc-MOG 35-55
MAILFAVVARGTTILAKHAWCGGNFLEVTEQILAKIPSENNKLTYSHGNYLFHYICQDRIVYLCITDDDFERSRAFNFLNEIKKRFQTTYGSRAQTALPYAMNSEFSSVLAAQLKHHSENKGLDKVMETQAQVDELKGIMVRNIDLVAQRGERLELLIDKTENLVDSSVTFKTTSRNLARAMCMKNLKLTIIIIIVSIVFIYIIVSPLCGGFTWPSCVKKSGGGGSGGGGSGGGGSRRARRMEVGWYRSPFSRVVHLYRNGKMEVGWYRSPFSRVVHLYRNGKMEVGWYRSPFSRVVHLYRNGKMEVGWYRSPFSRVVHLYRNGKMEVGWYRSPFSRVVHLYRNGKMEVGWYRSPFSRVVHLYRNGKMEVGWYRSPFSRVVHLYRNGK

SEQ ID NO: 106 - protein, 4 aa, synthetic construct
  REGION >4: note = The entire sequences of amino acids 1-4 can be repeated one to five times.
GGGS

SEQ ID NO: 107 - protein, 5 aa, synthetic construct
  REGION >5: note = The entire sequences of amino acids 1-5 can be repeated one to five times.
GGGGS

SEQ ID NO: 108 - protein, 5 aa, synthetic construct
  REGION >5: note = The entire sequences of amino acids 1-5 can be repeated one to five times.
EAAAK